European Patent Application EP 4 183 412 A1, published May 24, 2023. Title: RSV F PROTEIN COMPOSITIONS AND METHODS FOR MAKING SAME. Applicant: GlaxoSmithKline Biologicals S.A. The sequence listing filed with the application follows.

SEQUENCE LISTING (112 sequences)

SEQ ID NO: 1 - protein, 574 aa, Human respiratory syncytial virus
MELLILKANAITTILTAVTFCFASGQNITEEFYQSTCSAVSKGYLSALRTGWYTSVITIELSNIKENKCNGTDAKVKLIKQELDKYKNAVTELQLLMQSTPPTNNRARRELPRFMNYTLNNAKKTNVTLSKKRKRRFLGFLLGVGSAIASGVAVSKVLHLEGEVNKIKSALLSTNKAVVSLSNGVSVLTSKVLDLKNYIDKQLLPIVNKQSCSISNIETVIEFQQKNNRLLEITREFSVNAGVTTPVSTYMLTNSELLSLINDMPITNDQKKLMSNNVQIVRQQSYSIMSIIKEEVLAYVVQLPLYGVIDTPCWKLHTSPLCTTNTKEGSNICLTRTDRGWYCDNAGSVSFFPQAETCKVQSNRVFCDTMNSLTLPSEINLCNVDIFNPKYDCKIMTSKTDVSSSVITSLGAIVSCYGKTKCTASNKNRGIIKTFSNGCDYVSNKGMDTVSVGNTLYYVNKQEGKSLYVKGEPIINFYDPLVFPSDEFDASISQVNEKINQSLAFIRKSDELLHNVNAGKSTTNIMITTIIIVIIVILLSLIAVGLLLYCKARSTPVTLSKDQLSGINNIAFSN

SEQ ID NO: 2 - protein, 574 aa, Human respiratory syncytial virus
MELLIHRSSAIFLTLAVNALYLTSSQNITEEFYQSTCSAVSRGYFSALRTGWYTSVITIELSNIKETKCNGTDTKVKLIKQELDKYKNAVTELQLLMQNTPAANNRARREAPQYMNYTINTTKNLNVSISKKRKRRFLGFLLGVGSAIASGIAVSKVLHLEGEVNKIKNALLSTNKAVVSLSNGVSVLTSKVLDLKNYINNRLLPIVNQQSCRISNIETVIEFQQMNSRLLEITREFSVNAGVTTPLSTYMLTNSELLSLINDMPITNDQKKLMSSNVQIVRQQSYSIMSIIKEEVLAYVVQLPIYGVIDTPCWKLHTSPLCTTNIKEGSNICLTRTDRGWYCDNAGSVSFFPQADTCKVQSNRVFCDTMNSLTLPSEVSLCNTDIFNSKYDCKIMTSKTDISSSVITSLGAIVSCYGKTKCTASNKNRGIIKTFSNGCDYVSNKGVDTVSVGNTLYYVNKLEGKNLYVKGEPIINYYDPLVFPSDEFDASISQVNEKINQSLAFIRRSDELLHNVNTGKSTTNIMITTIIIVIIVVLLSLIAIGLLLYCKAKNTPVTLSKDQLSGINNIAFSK

SEQ ID NO: 3 - protein, 51 aa, synthetic construct
  REGION 1..51: note = Description of Artificial Sequence: Syntheticpolypeptide
TPATNNRARKELPRFMNYTLNNAKKTNVTLSKKRKKKFLGFLLGVGSAIAS

SEQ ID NO: 4 - protein, 48 aa, synthetic construct
  REGION 1..48: note = Description of Artificial Sequence: Syntheticpolypeptide
TPATNNRARQELPRFMNYTLNNAKKTNVTLSKKRFLGFLLGVGSAIAS

SEQ ID NO: 5 - protein, 51 aa, synthetic construct
  REGION 1..51: note = Description of Artificial Sequence: Syntheticpolypeptide
TPATNNQAQNELPQFMNYTLNNANNTNVTLSQNQNQNFLGFLLGVGSAIAS

SEQ ID NO: 6 - protein, 51 aa, synthetic construct
  REGION 1..51: note = Description of Artificial Sequence: Syntheticpolypeptide
TPATNNQAQNELPRFMNYTLNNAKKTNVTLSQNQNQNFLGFLLGVGSAIAS

SEQ ID NO: 7 - protein, 30 aa, synthetic construct
  REGION 1..30: note = Description of Artificial Sequence: Syntheticpolypeptide
TPATNNQAQNQNQNQNFLGFLLGVGSAIAS

SEQ ID NO: 8 - protein, 28 aa, synthetic construct
  REGION 1..28: note = Description of Artificial Sequence: Syntheticpeptide
TPATNNQAQNQNQNFLGFLLGVGSAIAS

SEQ ID NO: 9 - protein, 28 aa, synthetic construct
  REGION 1..28: note = Description of Artificial Sequence: Syntheticpeptide
TPATNNRARQQQQRFLGFLLGVGSAIAS

SEQ ID NO: 10 - protein, 51 aa, synthetic construct
  REGION 1..51: note = Description of Artificial Sequence: Syntheticpolypeptide
TPATNNRARRELPQFMNYTLNNAQQTNVTLSQNQNQNFLGFLLGVGSAIAS

SEQ ID NO: 11 - protein, 51 aa, synthetic construct
  REGION 1..51: note = Description of Artificial Sequence: Syntheticpolypeptide
TPATNNQAQNELPQFMNYTLNNAQQTNVTLSKKRKRRFLGFLLGVGSAIAS

SEQ ID NO: 12 - protein, 42 aa, synthetic construct
  REGION 1..42: note = Description of Artificial Sequence: Syntheticpolypeptide
TPATNNRARRELPRFMNYTLNNAKKTNVTLSKKRKRRSAIAS

SEQ ID NO: 13 - protein, 51 aa, synthetic construct
  REGION 1..51: note = Description of Artificial Sequence: Syntheticpolypeptide
TPATNNIEGRELPRFMNYTLNNAKKTNVTLSKKIEGRFLGFLLGVGSAIAS

SEQ ID NO: 14 - protein, 64 aa, synthetic construct
  REGION 1..64: note = Description of Artificial Sequence: Syntheticpolypeptide
PLVFPSDEFDASISQVNEKINQSLAFIRKSDELLHNVNDKIEEILSKIYHIENEIARIKKLIGE

SEQ ID NO: 15 - protein, 60 aa, synthetic construct
  REGION 1..60: note = Description of Artificial Sequence: Syntheticpolypeptide
PLVFPSDEFDASISQVNEKINQSLAFIRKSDELLHNVNEKFHQIEKEFSEVEGRIQDLEK

SEQ ID NO: 16 - protein, 38 aa, synthetic construct
  REGION 1..38: note = Description of Artificial Sequence: Syntheticpolypeptide
PLVFPSDEFDASISQINEKINQILAFIRKIDELLHNIN

SEQ ID NO: 17 - protein, 67 aa, synthetic construct
  REGION 1..67: note = Description of Artificial Sequence: Syntheticpolypeptide
PLVFPSDEFDASISQVNEKINQSLAFIRKSDELLHNVNGSGYIPEAPRDGQAYVRKDGEWVLLSTFL

SEQ ID NO: 18 - protein, 73 aa, synthetic construct
  REGION 1..73: note = Description of Artificial Sequence: Syntheticpolypeptide
PLVFPSDEFDASISQVNEKINQSLAFIRKSDELLHNVNNKNDDKGSGYIPEAPRDGQAYVRKDGEWVLLSTFL

SEQ ID NO: 19 - protein, 29 aa, unidentified
  REGION 1..29: note = Description of Unknown:Bacteriophage T4 fibritin sequence
GSGYIPEAPRDGQAYVRKDGEWVLLSTFL

SEQ ID NO: 20 - protein, 31 aa, synthetic construct
  REGION 1..31: note = Description of Artificial Sequence: Syntheticpolypeptide
KQIEDKIEEILSKIYHIENEIARIKKLIGEA

SEQ ID NO: 21 - protein, 574 aa, Human respiratory syncytial virus
MELLILKANAITTILTAVTFCFASGQNITEEFYQSTCSAVSKGYLSALRTGWYTSVITIELSNIKENKCNGTDAKVKLIKQELDKYKNAVTELQLLMQSTPATNNRARRELPRFMNYTLNNAKKTNVTLSKKRKRRFLGFLLGVGSAIASGVAVSKVLHLEGEVNKIKSALLSTNKAVVSLSNGVSVLTSKVLDLKNYIDKQLLPIVNKQSCSISNIETVIEFQQKNNRLLEITREFSVNAGVTTPVSTYMLTNSELLSLINDMPITNDQKKLMSNNVQIVRQQSYSIMSIIKEEVLAYVVQLPLYGVIDTPCWKLHTSPLCTTNTKEGSNICLTRTDRGWYCDNAGSVSFFPQAETCKVQSNRVFCDTMNSLTLPSEVNLCNVDIFNPKYDCKIMTSKTDVSSSVITSLGAIVSCYGKTKCTASNKNRGIIKTFSNGCDYVSNKGVDTVSVGNTLYYVNKQEGKSLYVKGEPIINFYDPLVFPSDEFDASISQVNEKINQSLAFIRKSDELLHNVNAGKSTTNIMITTIIIVIIVILLSLIAVGLLLYCKARSTPVTLSKDQLSGINNIAFSN

SEQ ID NO: 22 - DNA, 1727 bp, Human respiratory syncytial virus
  source 1..1727: mol_type = genomic DNA
atggaactgctgatcctgaaggccaacgccatcaccaccatcctgaccgccgtgaccttctgcttcgccagcggccagaacatcaccgaggaattctaccagagcacctgcagcgccgtgagcaagggctacctgagcgccctgcggaccggctggtacaccagcgtgatcaccatcgagctgtccaacatcaaagaaaacaagtgcaacggcaccgacgccaaggtgaaactgatcaagcaggaactggacaagtacaagaacgccgtgaccgagctgcagctgctgatgcagagcacccccgccaccaacaaccgggccagaagagagctgccccggttcatgaactacaccctgaacaacgccaagaaaaccaacgtgaccctgagcaagaagcggaagcggcggttcctgggcttcctgctgggcgtgggcagcgccatcgccagcggggtggccgtgtccaaggtgctgcacctggaaggcgaggtgaacaagatcaagtccgccctgctgtccaccaacaaggccgtggtgtccctgagcaacggcgtgagcgtgctgaccagcaaggtgctggatctgaagaactacatcgacaagcagctgctgcccatcgtgaacaagcagagctgcagcatcagcaacatcgagaccgtgatcgagttccagcagaagaacaaccggctgctggaaatcacccgggagttcagcgtgaacgccggcgtgaccacccccgtgagcacctacatgctgaccaacagcgagctgctgtccctgatcaatgacatgcccatcaccaacgaccagaaaaagctgatgagcaacaacgtgcagatcgtgcggcagcagagctactccatcatgagcatcatcaaagaagaggtgctggcctacgtggtgcagctgcccctgtacggcgtgatcgacaccccctgctggaagctgcacaccagccccctgtgcaccaccaacaccaaagagggcagcaacatctgcctgacccggaccgaccggggctggtactgcgacaacgccggcagcgtgagcttcttcccccaagccgagacctgcaaggtgcagagcaaccgggtgttctgcgacaccatgaacagcctgaccctgccctccgaggtgaacctgtgcaacgtggacatcttcaaccccaagtacgactgcaagatcatgacctccaagaccgacgtgagcagctccgtgatcacctccctgggcgccatcgtgagctgctacggcaagaccaagtgcaccgccagcaacaagaaccggggcatcatcaagaccttcagcaacggctgcgactacgtgagcaacaagggcgtggacaccgtgagcgtgggcaacacactgtactacgtgaataagcaggaaggcaagagcctgtacgtgaagggcgagcccatcatcaacttctacgaccccctggtgttccccagcgacgagttcgacgccagcatcagccaggtcaacgagaagatcaaccagagcctggccttcatccggaagagcgacgagctgctgcacaatgtgaatgccggcaagagcaccaccaatatcatgatcaccacaatcatcatcgtgatcattgtgatcctgctgtctctgattgccgtgggcctgctgctgtactgcaaggcccgcagcacccctgtgaccctgtccaaggaccagctgtccggcatcaacaatatcgccttctccaactgaag

SEQ ID NO: 23 - protein, 588 aa, synthetic construct
  REGION 1..588: note = Description of Artificial Sequence: Syntheticpolypeptide
MELLILKANAITTILTAVTFCFASGQNITEEFYQSTCSAVSKGYLSALRTGWYTSVITIELSNIKENKCNGTDAKVKLIKQELDKYKNAVTELQLLMQSTPATNNRARRELPRFMNYTLNNAKKTNVTLSKKRKRRFLGFLLGVGSAIASGVAVSKVLHLEGEVNKIKSALLSTNKAVVSLSNGVSVLTSKVLDLKNYIDKQLLPIVNKQSCSISNIETVIEFQQKNNRLLEITREFSVNAGVTTPVSTYMLTNSELLSLINDMPITNDQKKLMSNNVQIVRQQSYSIMSIIKEEVLAYVVQLPLYGVIDTPCWKLHTSPLCTTNTKEGSNICLTRTDRGWYCDNAGSVSFFPQAETCKVQSNRVFCDTMNSLTLPSEVNLCNVDIFNPKYDCKIMTSKTDVSSSVITSLGAIVSCYGKTKCTASNKNRGIIKTFSNGCDYVSNKGVDTVSVGNTLYYVNKQEGKSLYVKGEPIINFYDPLVFPSDEFDASISQVNEKINQSLAFIRKSDELLHNVNAGKSTTNIMITTIIIVIIVILLSLIAVGLLLYCKARSTPVTLSKDQLSGINNIAFSNSGGSAGSGHHHHHH

SEQ ID NO: 24 - DNA, 1769 bp, synthetic construct
  misc_feature 1..1769: note = Description of Artificial Sequence: Syntheticpolynucleotide
  source 1..1769: mol_type = other DNA
atggaactgctgatcctgaaggccaacgccatcaccaccatcctgaccgccgtgaccttctgcttcgccagcggccagaacatcaccgaggaattctaccagagcacctgcagcgccgtgagcaagggctacctgagcgccctgcggaccggctggtacaccagcgtgatcaccatcgagctgtccaacatcaaagaaaacaagtgcaacggcaccgacgccaaggtgaaactgatcaagcaggaactggacaagtacaagaacgccgtgaccgagctgcagctgctgatgcagagcacccccgccaccaacaaccgggccagaagagagctgccccggttcatgaactacaccctgaacaacgccaagaaaaccaacgtgaccctgagcaagaagcggaagcggcggttcctgggcttcctgctgggcgtgggcagcgccatcgccagcggggtggccgtgtccaaggtgctgcacctggaaggcgaggtgaacaagatcaagtccgccctgctgtccaccaacaaggccgtggtgtccctgagcaacggcgtgagcgtgctgaccagcaaggtgctggatctgaagaactacatcgacaagcagctgctgcccatcgtgaacaagcagagctgcagcatcagcaacatcgagaccgtgatcgagttccagcagaagaacaaccggctgctggaaatcacccgggagttcagcgtgaacgccggcgtgaccacccccgtgagcacctacatgctgaccaacagcgagctgctgtccctgatcaatgacatgcccatcaccaacgaccagaaaaagctgatgagcaacaacgtgcagatcgtgcggcagcagagctactccatcatgagcatcatcaaagaagaggtgctggcctacgtggtgcagctgcccctgtacggcgtgatcgacaccccctgctggaagctgcacaccagccccctgtgcaccaccaacaccaaagagggcagcaacatctgcctgacccggaccgaccggggctggtactgcgacaacgccggcagcgtgagcttcttcccccaagccgagacctgcaaggtgcagagcaaccgggtgttctgcgacaccatgaacagcctgaccctgccctccgaggtgaacctgtgcaacgtggacatcttcaaccccaagtacgactgcaagatcatgacctccaagaccgacgtgagcagctccgtgatcacctccctgggcgccatcgtgagctgctacggcaagaccaagtgcaccgccagcaacaagaaccggggcatcatcaagaccttcagcaacggctgcgactacgtgagcaacaagggcgtggacaccgtgagcgtgggcaacacactgtactacgtgaataagcaggaaggcaagagcctgtacgtgaagggcgagcccatcatcaacttctacgaccccctggtgttccccagcgacgagttcgacgccagcatcagccaggtcaacgagaagatcaaccagagcctggccttcatccggaagagcgacgagctgctgcacaatgtgaatgccggcaagagcaccaccaatatcatgatcaccacaatcatcatcgtgatcattgtgatcctgctgtctctgattgccgtgggcctgctgctgtactgcaaggcccgcagcacccctgtgaccctgtccaaggaccagctgtccggcatcaacaatatcgccttctccaacagcggcggcagcgccggctctggccaccaccaccatcaccactgaag

SEQ ID NO: 25 - protein, 624 aa, synthetic construct
  REGION 1..624: note = Description of Artificial Sequence: Syntheticpolypeptide
MELLILKANAITTILTAVTFCFASGQNITEEFYQSTCSAVSKGYLSALRTGWYTSVITIELSNIKENKCNGTDAKVKLIKQELDKYKNAVTELQLLMQSTPATNNRARRELPRFMNYTLNNAKKTNVTLSKKRKRRFLGFLLGVGSAIASGVAVSKVLHLEGEVNKIKSALLSTNKAVVSLSNGVSVLTSKVLDLKNYIDKQLLPIVNKQSCSISNIETVIEFQQKNNRLLEITREFSVNAGVTTPVSTYMLTNSELLSLINDMPITNDQKKLMSNNVQIVRQQSYSIMSIIKEEVLAYVVQLPLYGVIDTPCWKLHTSPLCTTNTKEGSNICLTRTDRGWYCDNAGSVSFFPQAETCKVQSNRVFCDTMNSLTLPSEVNLCNVDIFNPKYDCKIMTSKTDVSSSVITSLGAIVSCYGKTKCTASNKNRGIIKTFSNGCDYVSNKGVDTVSVGNTLYYVNKQEGKSLYVKGEPIINFYDPLVFPSDEFDASISQVNEKINQSLAFIRKSDELLHNVNAGKSTTNIMITTIIIVIIVILLSLIAVGLLLYCKARSTPVTLSKDQLSGINNIAFSNGSSGRMKQIEDKIEEILSKIYHIENEIARIKKLIGESGGSAGSGHHHHHH

SEQ ID NO: 26 - DNA, 1877 bp, synthetic construct
  misc_feature 1..1877: note = Description of Artificial Sequence: Syntheticpolynucleotide
  source 1..1877: mol_type = other DNA
atggaactgctgatcctgaaggccaacgccatcaccaccatcctgaccgccgtgaccttctgcttcgccagcggccagaacatcaccgaggaattctaccagagcacctgcagcgccgtgagcaagggctacctgagcgccctgcggaccggctggtacaccagcgtgatcaccatcgagctgtccaacatcaaagaaaacaagtgcaacggcaccgacgccaaggtgaaactgatcaagcaggaactggacaagtacaagaacgccgtgaccgagctgcagctgctgatgcagagcacccccgccaccaacaaccgggccagaagagagctgccccggttcatgaactacaccctgaacaacgccaagaaaaccaacgtgaccctgagcaagaagcggaagcggcggttcctgggcttcctgctgggcgtgggcagcgccatcgccagcggggtggccgtgtccaaggtgctgcacctggaaggcgaggtgaacaagatcaagtccgccctgctgtccaccaacaaggccgtggtgtccctgagcaacggcgtgagcgtgctgaccagcaaggtgctggatctgaagaactacatcgacaagcagctgctgcccatcgtgaacaagcagagctgcagcatcagcaacatcgagaccgtgatcgagttccagcagaagaacaaccggctgctggaaatcacccgggagttcagcgtgaacgccggcgtgaccacccccgtgagcacctacatgctgaccaacagcgagctgctgtccctgatcaatgacatgcccatcaccaacgaccagaaaaagctgatgagcaacaacgtgcagatcgtgcggcagcagagctactccatcatgagcatcatcaaagaagaggtgctggcctacgtggtgcagctgcccctgtacggcgtgatcgacaccccctgctggaagctgcacaccagccccctgtgcaccaccaacaccaaagagggcagcaacatctgcctgacccggaccgaccggggctggtactgcgacaacgccggcagcgtgagcttcttcccccaagccgagacctgcaaggtgcagagcaaccgggtgttctgcgacaccatgaacagcctgaccctgccctccgaggtgaacctgtgcaacgtggacatcttcaaccccaagtacgactgcaagatcatgacctccaagaccgacgtgagcagctccgtgatcacctccctgggcgccatcgtgagctgctacggcaagaccaagtgcaccgccagcaacaagaaccggggcatcatcaagaccttcagcaacggctgcgactacgtgagcaacaagggcgtggacaccgtgagcgtgggcaacacactgtactacgtgaataagcaggaaggcaagagcctgtacgtgaagggcgagcccatcatcaacttctacgaccccctggtgttccccagcgacgagttcgacgccagcatcagccaggtcaacgagaagatcaaccagagcctggccttcatccggaagagcgacgagctgctgcacaatgtgaatgccggcaagagcaccaccaatatcatgatcaccacaatcatcatcgtgatcattgtgatcctgctgtctctgattgccgtgggcctgctgctgtactgcaaggcccgcagcacccctgtgaccctgtccaaggaccagctgtccggcatcaacaatatcgccttctccaacggcagcagcggccggatgaagcagatcgaggacaagatcgaggaaatcctgagcaagatctaccacatcgagaacgagatcgcccggatcaagaagctgatcggcgaaagcggcggctctgccggaagcggccaccaccaccatcaccactgaag

SEQ ID NO: 27 - protein, 626 aa, synthetic construct
  REGION 1..626: note = Description of Artificial Sequence: Syntheticpolypeptide
MELLILKANAITTILTAVTFCFASGQNITEEFYQSTCSAVSKGYLSALRTGWYTSVITIELSNIKENKCNGTDAKVKLIKQELDKYKNAVTELQLLMQSTPATNNRARRELPRFMNYTLNNAKKTNVTLSKKRKRRFLGFLLGVGSAIASGVAVSKVLHLEGEVNKIKSALLSTNKAVVSLSNGVSVLTSKVLDLKNYIDKQLLPIVNKQSCSISNIETVIEFQQKNNRLLEITREFSVNAGVTTPVSTYMLTNSELLSLINDMPITNDQKKLMSNNVQIVRQQSYSIMSIIKEEVLAYVVQLPLYGVIDTPCWKLHTSPLCTTNTKEGSNICLTRTDRGWYCDNAGSVSFFPQAETCKVQSNRVFCDTMNSLTLPSEVNLCNVDIFNPKYDCKIMTSKTDVSSSVITSLGAIVSCYGKTKCTASNKNRGIIKTFSNGCDYVSNKGVDTVSVGNTLYYVNKQEGKSLYVKGEPIINFYDPLVFPSDEFDASISQVNEKINQSLAFIRKSDELLHNVNAGKSTTNIMITTIIIVIIVILLSLIAVGLLLYCKARSTPVTLSKDQLSGINNIAFSNGSSGSGRMKQIEDKIEEILSKIYHIENEIARIKKLIGESGGSAGSGHHHHHH

SEQ ID NO: 28 - DNA, 1883 bp, synthetic construct
  misc_feature 1..1883: note = Description of Artificial Sequence: Syntheticpolynucleotide
  source 1..1883: mol_type = other DNA
atggaactgctgatcctgaaggccaacgccatcaccaccatcctgaccgccgtgaccttctgcttcgccagcggccagaacatcaccgaggaattctaccagagcacctgcagcgccgtgagcaagggctacctgagcgccctgcggaccggctggtacaccagcgtgatcaccatcgagctgtccaacatcaaagaaaacaagtgcaacggcaccgacgccaaggtgaaactgatcaagcaggaactggacaagtacaagaacgccgtgaccgagctgcagctgctgatgcagagcacccccgccaccaacaaccgggccagaagagagctgccccggttcatgaactacaccctgaacaacgccaagaaaaccaacgtgaccctgagcaagaagcggaagcggcggttcctgggcttcctgctgggcgtgggcagcgccatcgccagcggggtggccgtgtccaaggtgctgcacctggaaggcgaggtgaacaagatcaagtccgccctgctgtccaccaacaaggccgtggtgtccctgagcaacggcgtgagcgtgctgaccagcaaggtgctggatctgaagaactacatcgacaagcagctgctgcccatcgtgaacaagcagagctgcagcatcagcaacatcgagaccgtgatcgagttccagcagaagaacaaccggctgctggaaatcacccgggagttcagcgtgaacgccggcgtgaccacccccgtgagcacctacatgctgaccaacagcgagctgctgtccctgatcaatgacatgcccatcaccaacgaccagaaaaagctgatgagcaacaacgtgcagatcgtgcggcagcagagctactccatcatgagcatcatcaaagaagaggtgctggcctacgtggtgcagctgcccctgtacggcgtgatcgacaccccctgctggaagctgcacaccagccccctgtgcaccaccaacaccaaagagggcagcaacatctgcctgacccggaccgaccggggctggtactgcgacaacgccggcagcgtgagcttcttcccccaagccgagacctgcaaggtgcagagcaaccgggtgttctgcgacaccatgaacagcctgaccctgccctccgaggtgaacctgtgcaacgtggacatcttcaaccccaagtacgactgcaagatcatgacctccaagaccgacgtgagcagctccgtgatcacctccctgggcgccatcgtgagctgctacggcaagaccaagtgcaccgccagcaacaagaaccggggcatcatcaagaccttcagcaacggctgcgactacgtgagcaacaagggcgtggacaccgtgagcgtgggcaacacactgtactacgtgaataagcaggaaggcaagagcctgtacgtgaagggcgagcccatcatcaacttctacgaccccctggtgttccccagcgacgagttcgacgccagcatcagccaggtcaacgagaagatcaaccagagcctggccttcatccggaagagcgacgagctgctgcacaatgtgaatgccggcaagagcaccaccaatatcatgatcaccacaatcatcatcgtgatcattgtgatcctgctgtctctgattgccgtgggcctgctgctgtactgcaaggcccgcagcacccctgtgaccctgtccaaggaccagctgtccggcatcaacaatatcgccttctccaacggcagcagcggcagcggccggatgaagcagatcgaggacaagatcgaggaaatcctgagcaagatctaccacatcgagaacgagatcgcccggatcaagaagctgatcggcgaaagcggcggctctgccggaagcggccaccaccaccatcaccactgaag

SEQ ID NO: 29 - protein, 531 aa, synthetic construct
  REGION 1..531: note = Description of Artificial Sequence: Syntheticpolypeptide
MELLILKANAITTILTAVTFCFASGQNITEEFYQSTCSAVSKGYLSALRTGWYTSVITIELSNIKENKCNGTDAKVKLIKQELDKYKNAVTELQLLMQSTPATNNRARRELPRFMNYTLNNAKKTNVTLSKKRKRRFLGFLLGVGSAIASGVAVSKVLHLEGEVNKIKSALLSTNKAVVSLSNGVSVLTSKVLDLKNYIDKQLLPIVNKQSCSISNIETVIEFQQKNNRLLEITREFSVNAGVTTPVSTYMLTNSELLSLINDMPITNDQKKLMSNNVQIVRQQSYSIMSIIKEEVLAYVVQLPLYGVIDTPCWKLHTSPLCTTNTKEGSNICLTRTDRGWYCDNAGSVSFFPQAETCKVQSNRVFCDTMNSLTLPSEVNLCNVDIFNPKYDCKIMTSKTDVSSSVITSLGAIVSCYGKTKCTASNKNRGIIKTFSNGCDYVSNKGVDTVSVGNTLYYVNKQEGKSLYVKGEPIINFYDPLVFPSDEFDASISQVNEKINQSLAFIRKSDELLHNVNSGGSAGSGHHHHHH

SEQ ID NO: 30 - DNA, 1598 bp, synthetic construct
  misc_feature 1..1598: note = Description of Artificial Sequence: Syntheticpolynucleotide
  source 1..1598: mol_type = other DNA
atggaactgctgatcctgaaggccaacgccatcaccaccatcctgaccgccgtgaccttctgcttcgccagcggccagaacatcaccgaggaattctaccagagcacctgcagcgccgtgagcaagggctacctgagcgccctgcggaccggctggtacaccagcgtgatcaccatcgagctgtccaacatcaaagaaaacaagtgcaacggcaccgacgccaaggtgaaactgatcaagcaggaactggacaagtacaagaacgccgtgaccgagctgcagctgctgatgcagagcacccccgccaccaacaaccgggccagaagagagctgccccggttcatgaactacaccctgaacaacgccaagaaaaccaacgtgaccctgagcaagaagcggaagcggcggttcctgggcttcctgctgggcgtgggcagcgccatcgccagcggggtggccgtgtccaaggtgctgcacctggaaggcgaggtgaacaagatcaagtccgccctgctgtccaccaacaaggccgtggtgtccctgagcaacggcgtgagcgtgctgaccagcaaggtgctggatctgaagaactacatcgacaagcagctgctgcccatcgtgaacaagcagagctgcagcatcagcaacatcgagaccgtgatcgagttccagcagaagaacaaccggctgctggaaatcacccgggagttcagcgtgaacgccggcgtgaccacccccgtgagcacctacatgctgaccaacagcgagctgctgtccctgatcaatgacatgcccatcaccaacgaccagaaaaagctgatgagcaacaacgtgcagatcgtgcggcagcagagctactccatcatgagcatcatcaaagaagaggtgctggcctacgtggtgcagctgcccctgtacggcgtgatcgacaccccctgctggaagctgcacaccagccccctgtgcaccaccaacaccaaagagggcagcaacatctgcctgacccggaccgaccggggctggtactgcgacaacgccggcagcgtgagcttcttcccccaagccgagacctgcaaggtgcagagcaaccgggtgttctgcgacaccatgaacagcctgaccctgccctccgaggtgaacctgtgcaacgtggacatcttcaaccccaagtacgactgcaagatcatgacctccaagaccgacgtgagcagctccgtgatcacctccctgggcgccatcgtgagctgctacggcaagaccaagtgcaccgccagcaacaagaaccggggcatcatcaagaccttcagcaacggctgcgactacgtgagcaacaagggcgtggacaccgtgagcgtgggcaacacactgtactacgtgaataagcaggaaggcaagagcctgtacgtgaagggcgagcccatcatcaacttctacgaccccctggtgttccccagcgacgagttcgacgccagcatcagccaggtcaacgagaagatcaaccagagcctggccttcatccggaagagcgacgagctgctgcacaatgtgaatagcggcggcagcgccggctctggccaccaccaccatcaccactgaag

SEQ ID NO: 31 - protein, 557 aa, synthetic construct
  REGION 1..557: note = Description of Artificial Sequence: Syntheticpolypeptide
MELLILKANAITTILTAVTFCFASGQNITEEFYQSTCSAVSKGYLSALRTGWYTSVITIELSNIKENKCNGTDAKVKLIKQELDKYKNAVTELQLLMQSTPATNNRARRELPRFMNYTLNNAKKTNVTLSKKRKRRFLGFLLGVGSAIASGVAVSKVLHLEGEVNKIKSALLSTNKAVVSLSNGVSVLTSKVLDLKNYIDKQLLPIVNKQSCSISNIETVIEFQQKNNRLLEITREFSVNAGVTTPVSTYMLTNSELLSLINDMPITNDQKKLMSNNVQIVRQQSYSIMSIIKEEVLAYVVQLPLYGVIDTPCWKLHTSPLCTTNTKEGSNICLTRTDRGWYCDNAGSVSFFPQAETCKVQSNRVFCDTMNSLTLPSEVNLCNVDIFNPKYDCKIMTSKTDVSSSVITSLGAIVSCYGKTKCTASNKNRGIIKTFSNGCDYVSNKGVDTVSVGNTLYYVNKQEGKSLYVKGEPIINFYDPLVFPSDEFDASISQVNEKINQSLAFIRKSDELLHNVNDKIEEILSKIYHIENEIARIKKLIGESGGSAGSGHHHHHH

SEQ ID NO: 32 - DNA, 1676 bp, synthetic construct
  misc_feature 1..1676: note = Description of Artificial Sequence: Syntheticpolynucleotide
  source 1..1676: mol_type = other DNA
atggaactgctgatcctgaaggccaacgccatcaccaccatcctgaccgccgtgaccttctgcttcgccagcggccagaacatcaccgaggaattctaccagagcacctgcagcgccgtgagcaagggctacctgagcgccctgcggaccggctggtacaccagcgtgatcaccatcgagctgtccaacatcaaagaaaacaagtgcaacggcaccgacgccaaggtgaaactgatcaagcaggaactggacaagtacaagaacgccgtgaccgagctgcagctgctgatgcagagcacccccgccaccaacaaccgggccagaagagagctgccccggttcatgaactacaccctgaacaacgccaagaaaaccaacgtgaccctgagcaagaagcggaagcggcggttcctgggcttcctgctgggcgtgggcagcgccatcgccagcggggtggccgtgtccaaggtgctgcacctggaaggcgaggtgaacaagatcaagtccgccctgctgtccaccaacaaggccgtggtgtccctgagcaacggcgtgagcgtgctgaccagcaaggtgctggatctgaagaactacatcgacaagcagctgctgcccatcgtgaacaagcagagctgcagcatcagcaacatcgagaccgtgatcgagttccagcagaagaacaaccggctgctggaaatcacccgggagttcagcgtgaacgccggcgtgaccacccccgtgagcacctacatgctgaccaacagcgagctgctgtccctgatcaatgacatgcccatcaccaacgaccagaaaaagctgatgagcaacaacgtgcagatcgtgcggcagcagagctactccatcatgagcatcatcaaagaagaggtgctggcctacgtggtgcagctgcccctgtacggcgtgatcgacaccccctgctggaagctgcacaccagccccctgtgcaccaccaacaccaaagagggcagcaacatctgcctgacccggaccgaccggggctggtactgcgacaacgccggcagcgtgagcttcttcccccaagccgagacctgcaaggtgcagagcaaccgggtgttctgcgacaccatgaacagcctgaccctgccctccgaggtgaacctgtgcaacgtggacatcttcaaccccaagtacgactgcaagatcatgacctccaagaccgacgtgagcagctccgtgatcacctccctgggcgccatcgtgagctgctacggcaagaccaagtgcaccgccagcaacaagaaccggggcatcatcaagaccttcagcaacggctgcgactacgtgagcaacaagggcgtggacaccgtgagcgtgggcaacacactgtactacgtgaataagcaggaaggcaagagcctgtacgtgaagggcgagcccatcatcaacttctacgaccccctggtgttccccagcgacgagttcgacgccagcatcagccaggtcaacgagaagatcaaccagagcctggccttcatccggaagagcgacgagctgctgcacaatgtgaatgacaagatcgaggaaatcctgagcaagatctaccacatcgagaacgagatcgcccggatcaagaagctgatcggcgaaagcggcggctctgccggaagcggccaccaccaccatcaccactgaag

SEQ ID NO: 33 - protein, 615 aa, synthetic construct
  REGION 1..615: note = Description of Artificial Sequence: Syntheticpolypeptide
MELLILKANAITTILTAVTFCFASGQNITEEFYQSTCSAVSKGYLSALRTGWYTSVITIELSNIKENKCNGTDAKVKLIKQELDKYKNAVTELQLLMQSTPATNNRARRELPRFMNYTLNNAKKTNVTLSKKRKRRFLGFLLGVGSAIASGVAVSKVLHLEGEVNKIKSALLSTNKAVVSLSNGVSVLTSKVLDLKNYIDKQLLPIVNKQSCSISNIETVIEFQQKNNRLLEITREFSVNAGVTTPVSTYMLTNSELLSLINDMPITNDQKKLMSNNVQIVRQQSYSIMSIIKEEVLAYVVQLPLYGVIDTPCWKLHTSPLCTTNTKEGSNICLTRTDRGWYCDNAGSVSFFPQAETCKVQSNRVFCDTMNSLTLPSEVNLCNVDIFNPKYDCKIMTSKTDVSSSVITSLGAIVSCYGKTKCTASNKNRGIIKTFSNGCDYVSNKGVDTVSVGNTLYYVNKQEGKSLYVKGEPIINFYDPLVFPSDEFDASISQVNEKINQSLAFIRKSDELLHNVNAGKSTTNIMITTIIIVIIVILLSLIAVGLLLYCKARSTPVTLSKDQLSGINNIAFSNGSSGNEKFHQIEKEFSEVEGRIQDLEKSGGSAGSGHHHHHH

SEQ ID NO: 34 - DNA, 1850 bp, synthetic construct
  misc_feature 1..1850: note = Description of Artificial Sequence: Syntheticpolynucleotide
  source 1..1850: mol_type = other DNA
atggaactgctgatcctgaaggccaacgccatcaccaccatcctgaccgccgtgaccttctgcttcgccagcggccagaacatcaccgaggaattctaccagagcacctgcagcgccgtgagcaagggctacctgagcgccctgcggaccggctggtacaccagcgtgatcaccatcgagctgtccaacatcaaagaaaacaagtgcaacggcaccgacgccaaggtgaaactgatcaagcaggaactggacaagtacaagaacgccgtgaccgagctgcagctgctgatgcagagcacccccgccaccaacaaccgggccagaagagagctgccccggttcatgaactacaccctgaacaacgccaagaaaaccaacgtgaccctgagcaagaagcggaagcggcggttcctgggcttcctgctgggcgtgggcagcgccatcgccagcggggtggccgtgtccaaggtgctgcacctggaaggcgaggtgaacaagatcaagtccgccctgctgtccaccaacaaggccgtggtgtccctgagcaacggcgtgagcgtgctgaccagcaaggtgctggatctgaagaactacatcgacaagcagctgctgcccatcgtgaacaagcagagctgcagcatcagcaacatcgagaccgtgatcgagttccagcagaagaacaaccggctgctggaaatcacccgggagttcagcgtgaacgccggcgtgaccacccccgtgagcacctacatgctgaccaacagcgagctgctgtccctgatcaatgacatgcccatcaccaacgaccagaaaaagctgatgagcaacaacgtgcagatcgtgcggcagcagagctactccatcatgagcatcatcaaagaagaggtgctggcctacgtggtgcagctgcccctgtacggcgtgatcgacaccccctgctggaagctgcacaccagccccctgtgcaccaccaacaccaaagagggcagcaacatctgcctgacccggaccgaccggggctggtactgcgacaacgccggcagcgtgagcttcttcccccaagccgagacctgcaaggtgcagagcaaccgggtgttctgcgacaccatgaacagcctgaccctgccctccgaggtgaacctgtgcaacgtggacatcttcaaccccaagtacgactgcaagatcatgacctccaagaccgacgtgagcagctccgtgatcacctccctgggcgccatcgtgagctgctacggcaagaccaagtgcaccgccagcaacaagaaccggggcatcatcaagaccttcagcaacggctgcgactacgtgagcaacaagggcgtggacaccgtgagcgtgggcaacacactgtactacgtgaataagcaggaaggcaagagcctgtacgtgaagggcgagcccatcatcaacttctacgaccccctggtgttccccagcgacgagttcgacgccagcatcagccaggtcaacgagaagatcaaccagagcctggccttcatccggaagagcgacgagctgctgcacaatgtgaatgccggcaagagcaccaccaatatcatgatcaccacaatcatcatcgtgatcattgtgatcctgctgtctctgattgccgtgggcctgctgctgtactgcaaggcccgcagcacccctgtgaccctgtccaaggaccagctgtccggcatcaacaatatcgccttctccaacggcagcagcggcaatgagaagttccaccagatcgagaaagaattcagcgaggtggagggccggatccaggacctggaaaagagcggcggctctgccggaagcggccaccaccaccatcaccactgaag

SEQ ID NO: 35 - protein, 553 aa, synthetic construct
  REGION 1..553: note = Description of Artificial Sequence: Syntheticpolypeptide
MELLILKANAITTILTAVTFCFASGQNITEEFYQSTCSAVSKGYLSALRTGWYTSVITIELSNIKENKCNGTDAKVKLIKQELDKYKNAVTELQLLMQSTPATNNRARRELPRFMNYTLNNAKKTNVTLSKKRKRRFLGFLLGVGSAIASGVAVSKVLHLEGEVNKIKSALLSTNKAVVSLSNGVSVLTSKVLDLKNYIDKQLLPIVNKQSCSISNIETVIEFQQKNNRLLEITREFSVNAGVTTPVSTYMLTNSELLSLINDMPITNDQKKLMSNNVQIVRQQSYSIMSIIKEEVLAYVVQLPLYGVIDTPCWKLHTSPLCTTNTKEGSNICLTRTDRGWYCDNAGSVSFFPQAETCKVQSNRVFCDTMNSLTLPSEVNLCNVDIFNPKYDCKIMTSKTDVSSSVITSLGAIVSCYGKTKCTASNKNRGIIKTFSNGCDYVSNKGVDTVSVGNTLYYVNKQEGKSLYVKGEPIINFYDPLVFPSDEFDASISQVNEKINQSLAFIRKSDELLHNVNEKFHQIEKEFSEVEGRIQDLEKSGGSAGSGHHHHHH

SEQ ID NO: 36 - DNA, 1664 bp, synthetic construct
  misc_feature 1..1664: note = Description of Artificial Sequence: Syntheticpolynucleotide
  source 1..1664: mol_type = other DNA
atggaactgctgatcctgaaggccaacgccatcaccaccatcctgaccgccgtgaccttctgcttcgccagcggccagaacatcaccgaggaattctaccagagcacctgcagcgccgtgagcaagggctacctgagcgccctgcggaccggctggtacaccagcgtgatcaccatcgagctgtccaacatcaaagaaaacaagtgcaacggcaccgacgccaaggtgaaactgatcaagcaggaactggacaagtacaagaacgccgtgaccgagctgcagctgctgatgcagagcacccccgccaccaacaaccgggccagaagagagctgccccggttcatgaactacaccctgaacaacgccaagaaaaccaacgtgaccctgagcaagaagcggaagcggcggttcctgggcttcctgctgggcgtgggcagcgccatcgccagcggggtggccgtgtccaaggtgctgcacctggaaggcgaggtgaacaagatcaagtccgccctgctgtccaccaacaaggccgtggtgtccctgagcaacggcgtgagcgtgctgaccagcaaggtgctggatctgaagaactacatcgacaagcagctgctgcccatcgtgaacaagcagagctgcagcatcagcaacatcgagaccgtgatcgagttccagcagaagaacaaccggctgctggaaatcacccgggagttcagcgtgaacgccggcgtgaccacccccgtgagcacctacatgctgaccaacagcgagctgctgtccctgatcaatgacatgcccatcaccaacgaccagaaaaagctgatgagcaacaacgtgcagatcgtgcggcagcagagctactccatcatgagcatcatcaaagaagaggtgctggcctacgtggtgcagctgcccctgtacggcgtgatcgacaccccctgctggaagctgcacaccagccccctgtgcaccaccaacaccaaagagggcagcaacatctgcctgacccggaccgaccggggctggtactgcgacaacgccggcagcgtgagcttcttcccccaagccgagacctgcaaggtgcagagcaaccgggtgttctgcgacaccatgaacagcctgaccctgccctccgaggtgaacctgtgcaacgtggacatcttcaaccccaagtacgactgcaagatcatgacctccaagaccgacgtgagcagctccgtgatcacctccctgggcgccatcgtgagctgctacggcaagaccaagtgcaccgccagcaacaagaaccggggcatcatcaagaccttcagcaacggctgcgactacgtgagcaacaagggcgtggacaccgtgagcgtgggcaacacactgtactacgtgaataagcaggaaggcaagagcctgtacgtgaagggcgagcccatcatcaacttctacgaccccctggtgttccccagcgacgagttcgacgccagcatcagccaggtcaacgagaagatcaaccagagcctggccttcatccggaagagcgacgagctgctgcacaatgtgaatgagaagttccaccagatcgagaaagaattcagcgaggtggagggccggatccaggacctggaaaagagcggcggctctgccggaagcggccaccaccaccatcaccactgaag

SEQ ID NO: 37 - protein, 534 aa, synthetic construct
  REGION 1..534: note = Description of Artificial Sequence: Syntheticpolypeptide
MELLILKANAITTILTAVTFCFASGQNITEEFYQSTCSAVSKGYLSALRTGWYTSVITIELSNIKENKCNGTDAKVKLIKQELDKYKNAVTELQLLMQSTPATNNRARRELPRFMNYTLNNAKKTNVTLSKKRKRRFLGFLLGVGSAIASGVAVSKVLHLEGEVNKIKSALLSTNKAVVSLSNGVSVLTSKVLDLKNYIDKQLLPIVNKQSCSISNIETVIEFQQKNNRLLEITREFSVNAGVTTPVSTYMLTNSELLSLINDMPITNDQKKLMSNNVQIVRQQSYSIMSIIKEEVLAYVVQLPLYGVIDTPCWKLHTSPLCTTNTKEGSNICLTRTDRGWYCDNAGSVSFFPQAETCKVQSNRVFCDTMNSLTLPSEVNLCNVDIFNPKYDCKIMTSKTDVSSSVITSLGAIVSCYGKTKCTASNKNRGIIKTFSNGCDYVSNKGVDTVSVGNTLYYVNKQEGKSLYVKGEPNIMITTIIIVIIVILLSLIAVGLLLYCKARSTPVTLSKDQLSGINNIAFSNMGGSHHHHHH

SEQ ID NO: 38 - DNA, 1607 bp, synthetic construct
  misc_feature 1..1607: note = Description of Artificial Sequence: Syntheticpolynucleotide
  source 1..1607: mol_type = other DNA
atggaactgctgatcctgaaggccaacgccatcaccaccatcctgaccgccgtgaccttctgcttcgccagcggccagaacatcaccgaggaattctaccagagcacctgcagcgccgtgagcaagggctacctgagcgccctgcggaccggctggtacaccagcgtgatcaccatcgagctgtccaacatcaaagaaaacaagtgcaacggcaccgacgccaaggtgaaactgatcaagcaggaactggacaagtacaagaacgccgtgaccgagctgcagctgctgatgcagagcacccccgccaccaacaaccgggccagaagagagctgccccggttcatgaactacaccctgaacaacgccaagaaaaccaacgtgaccctgagcaagaagcggaagcggcggttcctgggcttcctgctgggcgtgggcagcgccatcgccagcggggtggccgtgtccaaggtgctgcacctggaaggcgaggtgaacaagatcaagtccgccctgctgtccaccaacaaggccgtggtgtccctgagcaacggcgtgagcgtgctgaccagcaaggtgctggatctgaagaactacatcgacaagcagctgctgcccatcgtgaacaagcagagctgcagcatcagcaacatcgagaccgtgatcgagttccagcagaagaacaaccggctgctggaaatcacccgggagttcagcgtgaacgccggcgtgaccacccccgtgagcacctacatgctgaccaacagcgagctgctgtccctgatcaatgacatgcccatcaccaacgaccagaaaaagctgatgagcaacaacgtgcagatcgtgcggcagcagagctactccatcatgagcatcatcaaagaagaggtgctggcctacgtggtgcagctgcccctgtacggcgtgatcgacaccccctgctggaagctgcacaccagccccctgtgcaccaccaacaccaaagagggcagcaacatctgcctgacccggaccgaccggggctggtactgcgacaacgccggcagcgtgagcttcttcccccaagccgagacctgcaaggtgcagagcaaccgggtgttctgcgacaccatgaacagcctgaccctgccctccgaggtgaacctgtgcaacgtggacatcttcaaccccaagtacgactgcaagatcatgacctccaagaccgacgtgagcagctccgtgatcacctccctgggcgccatcgtgagctgctacggcaagaccaagtgcaccgccagcaacaagaaccggggcatcatcaagaccttcagcaacggctgcgactacgtgagcaacaagggcgtggacaccgtgagcgtgggcaacacactgtactacgtgaataagcaggaaggcaagagcctgtacgtgaagggcgagcccaatatcatgatcaccacaatcatcatcgtgatcattgtgatcctgctgtctctgattgccgtgggcctgctgctgtactgcaaggcccgcagcacccctgtgaccctgtccaaggaccagctgtccggcatcaacaatatcgccttctccaacatggggggttctcatcatcatcatcatcattgaag

SEQ ID NO: 39 - protein, 524 aa, synthetic construct
  REGION 1..524: note = Description of Artificial Sequence: Syntheticpolypeptide
MELLILKANAITTILTAVTFCFASGQNITEEFYQSTCSAVSKGYLSALRTGWYTSVITIELSNIKENKCNGTDAKVKLIKQELDKYKNAVTELQLLMQSTPATNNRARRELPRFMNYTLNNAKKTNVTLSKKRKRRFLGFLLGVGSAIASGVAVSKVLHLEGEVNKIKSALLSTNKAVVSLSNGVSVLTSKVLDLKNYIDKQLLPIVNKQSCSISNIETVIEFQQKNNRLLEITREFSVNAGVTTPVSTYMLTNSELLSLINDMPITNDQKKLMSNNVQIVRQQSYSIMSIIKEEVLAYVVQLPLYGVIDTPCWKLHTSPLCTTNTKEGSNICLTRTDRGWYCDNAGSVSFFPQAETCKVQSNRVFCDTMNSLTLPSEVNLCNVDIFNPKYDCKIMTSKTDVSSSVITSLGAIVSCYGKTKCTASNKNRGIIKTFSNGCDYVSNKGVDTVSVGNTLYYVNKQEGKSLYVKGEPIINFYDPLVFPSDEFDASISQVNEKINQSLAFIRKSDELLHNVNAGKSTTN

SEQ ID NO: 40 - DNA, 1577 bp, synthetic construct
  misc_feature 1..1577: note = Description of Artificial Sequence: Syntheticpolynucleotide
  source 1..1577: mol_type = other DNA
atggaactgctgatcctgaaggccaacgccatcaccaccatcctgaccgccgtgaccttctgcttcgccagcggccagaacatcaccgaggaattctaccagagcacctgcagcgccgtgagcaagggctacctgagcgccctgcggaccggctggtacaccagcgtgatcaccatcgagctgtccaacatcaaagaaaacaagtgcaacggcaccgacgccaaggtgaaactgatcaagcaggaactggacaagtacaagaacgccgtgaccgagctgcagctgctgatgcagagcacccccgccaccaacaaccgggccagaagagagctgccccggttcatgaactacaccctgaacaacgccaagaaaaccaacgtgaccctgagcaagaagcggaagcggcggttcctgggcttcctgctgggcgtgggcagcgccatcgccagcggggtggccgtgtccaaggtgctgcacctggaaggcgaggtgaacaagatcaagtccgccctgctgtccaccaacaaggccgtggtgtccctgagcaacggcgtgagcgtgctgaccagcaaggtgctggatctgaagaactacatcgacaagcagctgctgcccatcgtgaacaagcagagctgcagcatcagcaacatcgagaccgtgatcgagttccagcagaagaacaaccggctgctggaaatcacccgggagttcagcgtgaacgccggcgtgaccacccccgtgagcacctacatgctgaccaacagcgagctgctgtccctgatcaatgacatgcccatcaccaacgaccagaaaaagctgatgagcaacaacgtgcagatcgtgcggcagcagagctactccatcatgagcatcatcaaagaagaggtgctggcctacgtggtgcagctgcccctgtacggcgtgatcgacaccccctgctggaagctgcacaccagccccctgtgcaccaccaacaccaaagagggcagcaacatctgcctgacccggaccgaccggggctggtactgcgacaacgccggcagcgtgagcttcttcccccaagccgagacctgcaaggtgcagagcaaccgggtgttctgcgacaccatgaacagcctgaccctgccctccgaggtgaacctgtgcaacgtggacatcttcaaccccaagtacgactgcaagatcatgacctccaagaccgacgtgagcagctccgtgatcacctccctgggcgccatcgtgagctgctacggcaagaccaagtgcaccgccagcaacaagaaccggggcatcatcaagaccttcagcaacggctgcgactacgtgagcaacaagggcgtggacaccgtgagcgtgggcaacacactgtactacgtgaataagcaggaaggcaagagcctgtacgtgaagggcgagcccatcatcaacttctacgaccccctggtgttccccagcgacgagttcgacgccagcatcagccaggtcaacgagaagatcaaccagagcctggccttcatccggaagagcgacgagctgctgcacaatgtgaatgccggcaagagcaccaccaattgaag

SEQ ID NO: 41 - protein, 574 aa, Human respiratory syncytial virus; identical to SEQ ID NO: 21

SEQ ID NO: 42 - protein, 590 aa, synthetic construct
  REGION 1..590: note = Description of Artificial Sequence: Syntheticpolypeptide
MELLILKANAITTILTAVTFCFASGQNITEEFYQSTCSAVSKGYLSALRTGWYTSVITIELSNIKENKCNGTDAKVKLIKQELDKYKNAVTELQLLMQSTPATNNRARRELPRFMNYTLNNAKKTNVTLSKKRKRRFLGFLLGVGSAIASGVAVSKVLHLEGEVNKIKSALLSTNKAVVSLSNGVSVLTSKVLDLKNYIDKQLLPIVNKQSCSISNIETVIEFQQKNNRLLEITREFSVNAGVTTPVSTYMLTNSELLSLINDMPITNDQKKLMSNNVQIVRQQSYSIMSIIKEEVLAYVVQLPLYGVIDTPCWKLHTSPLCTTNTKEGSNICLTRTDRGWYCDNAGSVSFFPQAETCKVQSNRVFCDTMNSLTLPSEVNLCNVDIFNPKYDCKIMTSKTDVSSSVITSLGAIVSCYGKTKCTASNKNRGIIKTFSNGCDYVSNKGVDTVSVGNTLYYVNKQEGKSLYVKGEPIINFYDPLVFPSDEFDASISQINEKINQILAFIRKIDELLHNINAGKSTTNGSGSGDDDDDKGSGSGIMITTIIIVIIVILLSLIAVGLLLYCKARSTPVTLSKDQLSGINNIAFSN

SEQ ID NO: 43 - protein, 588 aa, synthetic construct
  REGION 1..588: note = Description of Artificial Sequence: Syntheticpolypeptide
MELLILKANAITTILTAVTFCFASGQNITEEFYQSTCSAVSKGYLSALRTGWYTSVITIELSNIKENKCNGTDAKVKLIKQELDKYKNAVTELQLLMQSTPATNNRARRELPRFMNYTLNNAKKTNVTLSKKRKRRFLGFLLGVGSAIASGVAVSKVLHLEGEVNKIKSALLSTNKAVVSLSNGVSVLTSKVLDLKNYIDKQLLPIVNKQSCSISNIETVIEFQQKNNRLLEITREFSVNAGVTTPVSTYMLTNSELLSLINDMPITNDQKKLMSNNVQIVRQQSYSIMSIIKEEVLAYVVQLPLYGVIDTPCWKLHTSPLCTTNTKEGSNICLTRTDRGWYCDNAGSVSFFPQAETCKVQSNRVFCDTMNSLTLPSEVNLCNVDIFNPKYDCKIMTSKTDVSSSVITSLGAIVSCYGKTKCTASNKNRGIIKTFSNGCDYVSNKGVDTVSVGNTLYYVNKQEGKSLYVKGEPIINFYDPLVFPSDEFDASISQINEKINQILAFIRKIDELLHNINAGKSTTNGSGSGLVPRGSGSGIMITTIIIVIIVILLSLIAVGLLLYCKARSTPVTLSKDQLSGINNIAFSN

SEQ ID NO: 44 - protein, 588 aa, synthetic construct
  REGION 1..588: note = Description of Artificial Sequence: Syntheticpolypeptide
MELLILKANAITTILTAVTFCFASGQNITEEFYQSTCSAVSKGYLSALRTGWYTSVITIELSNIKENKCNGTDAKVKLIKQELDKYKNAVTELQLLMQSTPATNNRARRELPRFMNYTLNNAKKTNVTLSKKRKRRFLGFLLGVGSAIASGVAVSKVLHLEGEVNKIKSALLSTNKAVVSLSNGVSVLTSKVLDLKNYIDKQLLPIVNKQSCSISNIETVIEFQQKNNRLLEITREFSVNAGVTTPVSTYMLTNSELLSLINDMPITNDQKKLMSNNVQIVRQQSYSIMSIIKEEVLAYVVQLPLYGVIDTPCWKLHTSPLCTTNTKEGSNICLTRTDRGWYCDNAGSVSFFPQAETCKVQSNRVFCDTMNSLTLPSEVNLCNVDIFNPKYDCKIMTSKTDVSSSVITSLGAIVSCYGKTKCTASNKNRGIIKTFSNGCDYVSNKGVDTVSVGNTLYYVNKQEGKSLYVKGEPIINFYDPLVFPSDEFDASISQINEKINQILAFIRKIDELLHNINAGKSTTNGSGSGIEGRGSGSGIMITTIIIVIIVILLSLIAVGLLLYCKARSTPVTLSKDQLSGINNIAFSN

SEQ ID NO: 45 - protein, 537 aa, synthetic construct
  REGION 1..537: note = Description of Artificial Sequence: Syntheticpolypeptide
MELLILKANAITTILTAVTFCFASGQNITEEFYQSTCSAVSKGYLSALRTGWYTSVITIELSNIKENKCNGTDAKVKLIKQELDKYKNAVTELQLLMQSTPATNNQAQNELPRFMNYTLNNAKKTNVTLSQNQNQNFLGFLLGVGSAIASGVAVSKVLHLEGEVNKIKSALLSTNKAVVSLSNGVSVLTSKVLDLKNYIDKQLLPIVNKQSCSISNIETVIEFQQKNNRLLEITREFSVNAGVTTPVSTYMLTNSELLSLINDMPITNDQKKLMSNNVQIVRQQSYSIMSIIKEEVLAYVVQLPLYGVIDTPCWKLHTSPLCTTNTKEGSNICLTRTDRGWYCDNAGSVSFFPQAETCKVQSNRVFCDTMNSLTLPSEVNLCNVDIFNPKYDCKIMTSKTDVSSSVITSLGAIVSCYGKTKCTASNKNRGIIKTFSNGCDYVSNKGVDTVSVGNTLYYVNKQEGKSLYVKGEPIINFYDPLVFPSDEFDASISQVNEKINQSLAFIRKSDELLHNVNAGKSTTNGGSAGSGHHHHHH

SEQ ID NO: 46 - protein, 537 aa, synthetic construct
  REGION 1..537: note = Description of Artificial Sequence: Syntheticpolypeptide
MELLILKANAITTILTAVTFCFASGQNITEEFYQSTCSAVSKGYLSALRTGWYTSVITIELSNIKENKCNGTDAKVKLIKQELDKYKNAVTELQLLMQSTPATNNQAQNELPQFMNYTLNNANNTNVTLSQNQNQNFLGFLLGVGSAIASGVAVSKVLHLEGEVNKIKSALLSTNKAVVSLSNGVSVLTSKVLDLKNYIDKQLLPIVNKQSCSISNIETVIEFQQKNNRLLEITREFSVNAGVTTPVSTYMLTNSELLSLINDMPITNDQKKLMSNNVQIVRQQSYSIMSIIKEEVLAYVVQLPLYGVIDTPCWKLHTSPLCTTNTKEGSNICLTRTDRGWYCDNAGSVSFFPQAETCKVQSNRVFCDTMNSLTLPSEVNLCNVDIFNPKYDCKIMTSKTDVSSSVITSLGAIVSCYGKTKCTASNKNRGIIKTFSNGCDYVSNKGVDTVSVGNTLYYVNKQEGKSLYVKGEPIINFYDPLVFPSDEFDASISQVNEKINQSLAFIRKSDELLHNVNAGKSTTNGGSAGSGHHHHHH

SEQ ID NO: 47 - protein, 516 aa, synthetic construct
  REGION 1..516: note = Description of Artificial Sequence: Syntheticpolypeptide
MELLILKANAITTILTAVTFCFASGQNITEEFYQSTCSAVSKGYLSALRTGWYTSVITIELSNIKENKCNGTDAKVKLIKQELDKYKNAVTELQLLMQSTPATNNQAQNQNQNQNFLGFLLGVGSAIASGVAVSKVLHLEGEVNKIKSALLSTNKAVVSLSNGVSVLTSKVLDLKNYIDKQLLPIVNKQSCSISNIETVIEFQQKNNRLLEITREFSVNAGVTTPVSTYMLTNSELLSLINDMPITNDQKKLMSNNVQIVRQQSYSIMSIIKEEVLAYVVQLPLYGVIDTPCWKLHTSPLCTTNTKEGSNICLTRTDRGWYCDNAGSVSFFPQAETCKVQSNRVFCDTMNSLTLPSEVNLCNVDIFNPKYDCKIMTSKTDVSSSVITSLGAIVSCYGKTKCTASNKNRGIIKTFSNGCDYVSNKGVDTVSVGNTLYYVNKQEGKSLYVKGEPIINFYDPLVFPSDEFDASISQVNEKINQSLAFIRKSDELLHNVNAGKSTTNGGSAGSGHHHHHH

SEQ ID NO: 48 - protein, 514 aa, synthetic construct
  REGION 1..514: note = Description of Artificial Sequence: Syntheticpolypeptide
MELLILKANAITTILTAVTFCFASGQNITEEFYQSTCSAVSKGYLSALRTGWYTSVITIELSNIKENKCNGTDAKVKLIKQELDKYKNAVTELQLLMQSTPATNNQAQNQNQNFLGFLLGVGSAIASGVAVSKVLHLEGEVNKIKSALLSTNKAVVSLSNGVSVLTSKVLDLKNYIDKQLLPIVNKQSCSISNIETVIEFQQKNNRLLEITREFSVNAGVTTPVSTYMLTNSELLSLINDMPITNDQKKLMSNNVQIVRQQSYSIMSIIKEEVLAYVVQLPLYGVIDTPCWKLHTSPLCTTNTKEGSNICLTRTDRGWYCDNAGSVSFFPQAETCKVQSNRVFCDTMNSLTLPSEVNLCNVDIFNPKYDCKIMTSKTDVSSSVITSLGAIVSCYGKTKCTASNKNRGIIKTFSNGCDYVSNKGVDTVSVGNTLYYVNKQEGKSLYVKGEPIINFYDPLVFPSDEFDASISQVNEKINQSLAFIRKSDELLHNVNAGKSTTNGGSAGSGHHHHHH

SEQ ID NO: 49 - protein, 514 aa, synthetic construct
  REGION 1..514: note = Description of Artificial Sequence: Syntheticpolypeptide
MELLILKANAITTILTAVTFCFASGQNITEEFYQSTCSAVSKGYLSALRTGWYTSVITIELSNIKENKCNGTDAKVKLIKQELDKYKNAVTELQLLMQSTPATNNRARQQQQRFLGFLLGVGSAIASGVAVSKVLHLEGEVNKIKSALLSTNKAVVSLSNGVSVLTSKVLDLKNYIDKQLLPIVNKQSCSISNIETVIEFQQKNNRLLEITREFSVNAGVTTPVSTYMLTNSELLSLINDMPITNDQKKLMSNNVQIVRQQSYSIMSIIKEEVLAYVVQLPLYGVIDTPCWKLHTSPLCTTNTKEGSNICLTRTDRGWYCDNAGSVSFFPQAETCKVQSNRVFCDTMNSLTLPSEVNLCNVDIFNPKYDCKIMTSKTDVSSSVITSLGAIVSCYGKTKCTASNKNRGIIKTFSNGCDYVSNKGVDTVSVGNTLYYVNKQEGKSLYVKGEPIINFYDPLVFPSDEFDASISQVNEKINQSLAFIRKSDELLHNVNAGKSTTNGGSAGSGHHHHHH

SEQ ID NO: 50 - protein, 537 aa, synthetic construct
  REGION 1..537: note = Description of Artificial Sequence: Syntheticpolypeptide
MELLILKANAITTILTAVTFCFASGQNITEEFYQSTCSAVSKGYLSALRTGWYTSVITIELSNIKENKCNGTDAKVKLIKQELDKYKNAVTELQLLMQSTPATNNRARKELPRFMNYTLNNAKKTNVTLSKKRKKKFLGFLLGVGSAIASGVAVSKVLHLEGEVNKIKSALLSTNKAVVSLSNGVSVLTSKVLDLKNYIDKQLLPIVNKQSCSISNIETVIEFQQKNNRLLEITREFSVNAGVTTPVSTYMLTNSELLSLINDMPITNDQKKLMSNNVQIVRQQSYSIMSIIKEEVLAYVVQLPLYGVIDTPCWKLHTSPLCTTNTKEGSNICLTRTDRGWYCDNAGSVSFFPQAETCKVQSNRVFCDTMNSLTLPSEVNLCNVDIFNPKYDCKIMTSKTDVSSSVITSLGAIVSCYGKTKCTASNKNRGIIKTFSNGCDYVSNKGVDTVSVGNTLYYVNKQEGKSLYVKGEPIINFYDPLVFPSDEFDASISQVNEKINQSLAFIRKSDELLHNVNAGKSTTNGGSAGSGHHHHHH

SEQ ID NO: 51 - protein, 534 aa, synthetic construct
  REGION 1..534: note = Description of Artificial Sequence: Syntheticpolypeptide
MELLILKANAITTILTAVTFCFASGQNITEEFYQSTCSAVSKGYLSALRTGWYTSVITIELSNIKENKCNGTDAKVKLIKQELDKYKNAVTELQLLMQSTPATNNRARQELPRFMNYTLNNAKKTNVTLSKKRFLGFLLGVGSAIASGVAVSKVLHLEGEVNKIKSALLSTNKAVVSLSNGVSVLTSKVLDLKNYIDKQLLPIVNKQSCSISNIETVIEFQQKNNRLLEITREFSVNAGVTTPVSTYMLTNSELLSLINDMPITNDQKKLMSNNVQIVRQQSYSIMSIIKEEVLAYVVQLPLYGVIDTPCWKLHTSPLCTTNTKEGSNICLTRTDRGWYCDNAGSVSFFPQAETCKVQSNRVFCDTMNSLTLPSEVNLCNVDIFNPKYDCKIMTSKTDVSSSVITSLGAIVSCYGKTKCTASNKNRGIIKTFSNGCDYVSNKGVDTVSVGNTLYYVNKQEGKSLYVKGEPIINFYDPLVFPSDEFDASISQVNEKINQSLAFIRKSDELLHNVNAGKSTTNGGSAGSGHHHHHH

SEQ ID NO: 52 - protein, 537 aa, synthetic construct
  REGION 1..537: note = Description of Artificial Sequence: Syntheticpolypeptide
MELLILKANAITTILTAVTFCFASGQNITEEFYQSTCSAVSKGYLSALRTGWYTSVITIELSNIKENKCNGTDAKVKLIKQELDKYKNAVTELQLLMQSTPATNNIEGRELPRFMNYTLNNAKKTNVTLSKKIEGRFLGFLLGVGSAIASGVAVSKVLHLEGEVNKIKSALLSTNKAVVSLSNGVSVLTSKVLDLKNYIDKQLLPIVNKQSCSISNIETVIEFQQKNNRLLEITREFSVNAGVTTPVSTYMLTNSELLSLINDMPITNDQKKLMSNNVQIVRQQSYSIMSIIKEEVLAYVVQLPLYGVIDTPCWKLHTSPLCTTNTKEGSNICLTRTDRGWYCDNAGSVSFFPQAETCKVQSNRVFCDTMNSLTLPSEVNLCNVDIFNPKYDCKIMTSKTDVSSSVITSLGAIVSCYGKTKCTASNKNRGIIKTFSNGCDYVSNKGVDTVSVGNTLYYVNKQEGKSLYVKGEPIINFYDPLVFPSDEFDASISQVNEKINQSLAFIRKSDELLHNVNAGKSTTNGGSAGSGHHHHHH

SEQ ID NO: 53 - protein, 566 aa, synthetic construct
  REGION 1..566: note = Description of Artificial Sequence: Syntheticpolypeptide
MELLILKANAITTILTAVTFCFASGQNITEEFYQSTCSAVSKGYLSALRTGWYTSVITIELSNIKENKCNGTDAKVKLIKQELDKYKNAVTELQLLMQSTPATNNRARRELPRFMNYTLNNAKKTNVTLSKKRKRRFLGFLLGVGSAIASGVAVSKVLHLEGEVNKIKSALLSTNKAVVSLSNGVSVLTSKVLDLKNYIDKQLLPIVNKQSCSISNIETVIEFQQKNNRLLEITREFSVNAGVTTPVSTYMLTNSELLSLINDMPITNDQKKLMSNNVQIVRQQSYSIMSIIKEEVLAYVVQLPLYGVIDTPCWKLHTSPLCTTNTKEGSNICLTRTDRGWYCDNAGSVSFFPQAETCKVQSNRVFCDTMNSLTLPSEVNLCNVDIFNPKYDCKIMTSKTDVSSSVITSLGAIVSCYGKTKCTASNKNRGIIKTFSNGCDYVSNKGVDTVSVGNTLYYVNKQEGKSLYVKGEPIINFYDPLVFPSDEFDASISQVNEKINQSLAFIRKSDELLHNVNAGKSTTNGSGYIPEAPRDGQAYVRKDGEWVLLSTFLGGSAGSGHHHHHH

SEQ ID NO: 54 - protein, 572 aa, synthetic construct
  REGION 1..572: note = Description of Artificial Sequence: Syntheticpolypeptide
MELLILKANAITTILTAVTFCFASGQNITEEFYQSTCSAVSKGYLSALRTGWYTSVITIELSNIKENKCNGTDAKVKLIKQELDKYKNAVTELQLLMQSTPATNNRARRELPRFMNYTLNNAKKTNVTLSKKRKRRFLGFLLGVGSAIASGVAVSKVLHLEGEVNKIKSALLSTNKAVVSLSNGVSVLTSKVLDLKNYIDKQLLPIVNKQSCSISNIETVIEFQQKNNRLLEITREFSVNAGVTTPVSTYMLTNSELLSLINDMPITNDQKKLMSNNVQIVRQQSYSIMSIIKEEVLAYVVQLPLYGVIDTPCWKLHTSPLCTTNTKEGSNICLTRTDRGWYCDNAGSVSFFPQAETCKVQSNRVFCDTMNSLTLPSEVNLCNVDIFNPKYDCKIMTSKTDVSSSVITSLGAIVSCYGKTKCTASNKNRGIIKTFSNGCDYVSNKGVDTVSVGNTLYYVNKQEGKSLYVKGEPIINFYDPLVFPSDEFDASISQVNEKINQSLAFIRKSDELLHNVNAGKSTTNNKNDDKGSGYIPEAPRDGQAYVRKDGEWVLLSTFLGGSAGSGHHHHHH

SEQ ID NO: 55 - protein, 557 aa, synthetic construct; identical to SEQ ID NO: 31
  REGION 1..557: note = Description of Artificial Sequence: Syntheticpolypeptide

SEQ ID NO: 56 - protein, 553 aa, synthetic construct; identical to SEQ ID NO: 35
  REGION 1..553: note = Description of Artificial Sequence: Syntheticpolypeptide

SEQ ID NO: 57 - protein, 557 aa, synthetic construct
  REGION 1..557: note = Description of Artificial Sequence: Syntheticpolypeptide
MELLILKANAITTILTAVTFCFASGQNITEEFYQSTCSAVSKGYLSALRTGWYTSVITIELSNIKENKCNGTDAKVKLIKQELDKYKNAVTELQLLMQSTPATNNQAQNELPQFMNYTLNNANNTNVTLSQNQNQNFLGFLLGVGSAIASGVAVSKVLHLEGEVNKIKSALLSTNKAVVSLSNGVSVLTSKVLDLKNYIDKQLLPIVNKQSCSISNIETVIEFQQKNNRLLEITREFSVNAGVTTPVSTYMLTNSELLSLINDMPITNDQKKLMSNNVQIVRQQSYSIMSIIKEEVLAYVVQLPLYGVIDTPCWKLHTSPLCTTNTKEGSNICLTRTDRGWYCDNAGSVSFFPQAETCKVQSNRVFCDTMNSLTLPSEVNLCNVDIFNPKYDCKIMTSKTDVSSSVITSLGAIVSCYGKTKCTASNKNRGIIKTFSNGCDYVSNKGVDTVSVGNTLYYVNKQEGKSLYVKGEPIINFYDPLVFPSDEFDASISQVNEKINQSLAFIRKSDELLHNVNDKIEEILSKIYHIENEIARIKKLIGESGGSAGSGHHHHHH

SEQ ID NO: 58 - protein, 536 aa, synthetic construct
  REGION 1..536: note = Description of Artificial Sequence: Syntheticpolypeptide
MELLILKANAITTILTAVTFCFASGQNITEEFYQSTCSAVSKGYLSALRTGWYTSVITIELSNIKENKCNGTDAKVKLIKQELDKYKNAVTELQLLMQSTPATNNQAQNQNQNQNFLGFLLGVGSAIASGVAVSKVLHLEGEVNKIKSALLSTNKAVVSLSNGVSVLTSKVLDLKNYIDKQLLPIVNKQSCSISNIETVIEFQQKNNRLLEITREFSVNAGVTTPVSTYMLTNSELLSLINDMPITNDQKKLMSNNVQIVRQQSYSIMSIIKEEVLAYVVQLPLYGVIDTPCWKLHTSPLCTTNTKEGSNICLTRTDRGWYCDNAGSVSFFPQAETCKVQSNRVFCDTMNSLTLPSEVNLCNVDIFNPKYDCKIMTSKTDVSSSVITSLGAIVSCYGKTKCTASNKNRGIIKTFSNGCDYVSNKGVDTVSVGNTLYYVNKQEGKSLYVKGEPIINFYDPLVFPSDEFDASISQVNEKINQSLAFIRKSDELLHNVNDKIEEILSKIYHIENEIARIKKLIGESGGSAGSGHHHHHH

SEQ ID NO: 59 - protein, 534 aa, synthetic construct
  REGION 1..534: note = Description of Artificial Sequence: Syntheticpolypeptide
MELLILKANAITTILTAVTFCFASGQNITEEFYQSTCSAVSKGYLSALRTGWYTSVITIELSNIKENKCNGTDAKVKLIKQELDKYKNAVTELQLLMQSTPATNNQAQNQNQNFLGFLLGVGSAIASGVAVSKVLHLEGEVNKIKSALLSTNKAVVSLSNGVSVLTSKVLDLKNYIDKQLLPIVNKQSCSISNIETVIEFQQKNNRLLEITREFSVNAGVTTPVSTYMLTNSELLSLINDMPITNDQKKLMSNNVQIVRQQSYSIMSIIKEEVLAYVVQLPLYGVIDTPCWKLHTSPLCTTNTKEGSNICLTRTDRGWYCDNAGSVSFFPQAETCKVQSNRVFCDTMNSLTLPSEVNLCNVDIFNPKYDCKIMTSKTDVSSSVITSLGAIVSCYGKTKCTASNKNRGIIKTFSNGCDYVSNKGVDTVSVGNTLYYVNKQEGKSLYVKGEPIINFYDPLVFPSDEFDASISQVNEKINQSLAFIRKSDELLHNVNDKIEEILSKIYHIENEIARIKKLIGESGGSAGSGHHHHHH

SEQ ID NO: 60 - protein, 534 aa, synthetic construct
  REGION 1..534: note = Description of Artificial Sequence: Syntheticpolypeptide
MELLILKANAITTILTAVTFCFASGQNITEEFYQSTCSAVSKGYLSALRTGWYTSVITIELSNIKENKCNGTDAKVKLIKQELDKYKNAVTELQLLMQSTPATNNRARQQQQRFLGFLLGVGSAIASGVAVSKVLHLEGEVNKIKSALLSTNKAVVSLSNGVSVLTSKVLDLKNYIDKQLLPIVNKQSCSISNIETVIEFQQKNNRLLEITREFSVNAGVTTPVSTYMLTNSELLSLINDMPITNDQKKLMSNNVQIVRQQSYSIMSIIKEEVLAYVVQLPLYGVIDTPCWKLHTSPLCTTNTKEGSNICLTRTDRGWYCDNAGSVSFFPQAETCKVQSNRVFCDTMNSLTLPSEVNLCNVDIFNPKYDCKIMTSKTDVSSSVITSLGAIVSCYGKTKCTASNKNRGIIKTFSNGCDYVSNKGVDTVSVGNTLYYVNKQEGKSLYVKGEPIINFYDPLVFPSDEFDASISQVNEKINQSLAFIRKSDELLHNVNDKIEEILSKIYHIENEIARIKKLIGESGGSAGSGHHHHHH

SEQ ID NO: 61 - protein, 574 aa, synthetic construct
  REGION 1..574: note = Description of Artificial Sequence: Syntheticpolypeptide
MELLILKANAITTILTAVTFCFASGQNITEEFYQSTCSAVSKGYLSALRTGWYTSVITIELSNIKENKCNGTDAKVKLIKQELDKYKNAVTELQLLMQSTPATNNQAQNELPQFMNYTLNNANNTNVTLSQNQNQNFLGFLLGVGSAIASGVAVSKVLHLEGEVNKIKSALLSTNKAVVSLSNGVSVLTSKVLDLKNYIDKQLLPIVNKQSCSISNIETVIEFQQKNNRLLEITREFSVNAGVTTPVSTYMLTNSELLSLINDMPITNDQKKLMSNNVQIVRQQSYSIMSIIKEEVLAYVVQLPLYGVIDTPCWKLHTSPLCTTNTKEGSNICLTRTDRGWYCDNAGSVSFFPQAETCKVQSNRVFCDTMNSLTLPSEVNLCNVDIFNPKYDCKIMTSKTDVSSSVITSLGAIVSCYGKTKCTASNKNRGIIKTFSNGCDYVSNKGVDTVSVGNTLYYVNKQEGKSLYVKGEPIINFYDPLVFPSDEFDASISQVNEKINQSLAFIRKSDELLHNVNAGKSTTNIMITTIIIVIIVILLSLIAVGLLLYCKARSTPVTLSKDQLSGINNIAFSN

SEQ ID NO: 62 - protein, 553 aa, synthetic construct
  REGION 1..553: note = Description of Artificial Sequence: Syntheticpolypeptide
MELLILKANAITTILTAVTFCFASGQNITEEFYQSTCSAVSKGYLSALRTGWYTSVITIELSNIKENKCNGTDAKVKLIKQELDKYKNAVTELQLLMQSTPATNNQAQNQNQNQNFLGFLLGVGSAIASGVAVSKVLHLEGEVNKIKSALLSTNKAVVSLSNGVSVLTSKVLDLKNYIDKQLLPIVNKQSCSISNIETVIEFQQKNNRLLEITREFSVNAGVTTPVSTYMLTNSELLSLINDMPITNDQKKLMSNNVQIVRQQSYSIMSIIKEEVLAYVVQLPLYGVIDTPCWKLHTSPLCTTNTKEGSNICLTRTDRGWYCDNAGSVSFFPQAETCKVQSNRVFCDTMNSLTLPSEVNLCNVDIFNPKYDCKIMTSKTDVSSSVITSLGAIVSCYGKTKCTASNKNRGIIKTFSNGCDYVSNKGVDTVSVGNTLYYVNKQEGKSLYVKGEPIINFYDPLVFPSDEFDASISQVNEKINQSLAFIRKSDELLHNVNAGKSTTNIMITTIIIVIIVILLSLIAVGLLLYCKARSTPVTLSKDQLSGINNIAFSN

SEQ ID NO: 63 - protein, 551 aa, synthetic construct
  REGION 1..551: note = Description of Artificial Sequence: Syntheticpolypeptide
MELLILKANAITTILTAVTFCFASGQNITEEFYQSTCSAVSKGYLSALRTGWYTSVITIELSNIKENKCNGTDAKVKLIKQELDKYKNAVTELQLLMQSTPATNNQAQNQNQNFLGFLLGVGSAIASGVAVSKVLHLEGEVNKIKSALLSTNKAVVSLSNGVSVLTSKVLDLKNYIDKQLLPIVNKQSCSISNIETVIEFQQKNNRLLEITREFSVNAGVTTPVSTYMLTNSELLSLINDMPITNDQKKLMSNNVQIVRQQSYSIMSIIKEEVLAYVVQLPLYGVIDTPCWKLHTSPLCTTNTKEGSNICLTRTDRGWYCDNAGSVSFFPQAETCKVQSNRVFCDTMNSLTLPSEVNLCNVDIFNPKYDCKIMTSKTDVSSSVITSLGAIVSCYGKTKCTASNKNRGIIKTFSNGCDYVSNKGVDTVSVGNTLYYVNKQEGKSLYVKGEPIINFYDPLVFPSDEFDASISQVNEKINQSLAFIRKSDELLHNVNAGKSTTNIMITTIIIVIIVILLSLIAVGLLLYCKARSTPVTLSKDQLSGINNIAFSN

SEQ ID NO: 64 - protein, 551 aa, synthetic construct
  REGION 1..551: note = Description of Artificial Sequence: Syntheticpolypeptide
MELLILKANAITTILTAVTFCFASGQNITEEFYQSTCSAVSKGYLSALRTGWYTSVITIELSNIKENKCNGTDAKVKLIKQELDKYKNAVTELQLLMQSTPATNNRARQQQQRFLGFLLGVGSAIASGVAVSKVLHLEGEVNKIKSALLSTNKAVVSLSNGVSVLTSKVLDLKNYIDKQLLPIVNKQSCSISNIETVIEFQQKNNRLLEITREFSVNAGVTTPVSTYMLTNSELLSLINDMPITNDQKKLMSNNVQIVRQQSYSIMSIIKEEVLAYVVQLPLYGVIDTPCWKLHTSPLCTTNTKEGSNICLTRTDRGWYCDNAGSVSFFPQAETCKVQSNRVFCDTMNSLTLPSEVNLCNVDIFNPKYDCKIMTSKTDVSSSVITSLGAIVSCYGKTKCTASNKNRGIIKTFSNGCDYVSNKGVDTVSVGNTLYYVNKQEGKSLYVKGEPIINFYDPLVFPSDEFDASISQVNEKINQSLAFIRKSDELLHNVNAGKSTTNIMITTIIIVIIVILLSLIAVGLLLYCKARSTPVTLSKDQLSGINNIAFSN

SEQ ID NO: 65 - protein, 537 aa, synthetic construct
  REGION 1..537: note = Description of Artificial Sequence: Syntheticpolypeptide
MELLILKANAITTILTAVTFCFASGQNITEEFYQSTCSAVSKGYLSALRTGWYTSVITIELSNIKENKCNGTDAKVKLIKQELDKYKNAVTELQLLMQSTPATNNQAQNELPQFMNYTLNNAQQTNVTLSKKRKRRFLGFLLGVGSAIASGVAVSKVLHLEGEVNKIKSALLSTNKAVVSLSNGVSVLTSKVLDLKNYIDKQLLPIVNKQSCSISNIETVIEFQQKNNRLLEITREFSVNAGVTTPVSTYMLTNSELLSLINDMPITNDQKKLMSNNVQIVRQQSYSIMSIIKEEVLAYVVQLPLYGVIDTPCWKLHTSPLCTTNTKEGSNICLTRTDRGWYCDNAGSVSFFPQAETCKVQSNRVFCDTMNSLTLPSEVNLCNVDIFNPKYDCKIMTSKTDVSSSVITSLGAIVSCYGKTKCTASNKNRGIIKTFSNGCDYVSNKGVDTVSVGNTLYYVNKQEGKSLYVKGEPIINFYDPLVFPSDEFDASISQVNEKINQSLAFIRKSDELLHNVNAGKSTTNGGSAGSGHHHHHH

SEQ ID NO: 66 - protein, 537 aa, synthetic construct
  REGION 1..537: note = Description of Artificial Sequence: Syntheticpolypeptide
MELLILKANAITTILTAVTFCFASGQNITEEFYQSTCSAVSKGYLSALRTGWYTSVITIELSNIKENKCNGTDAKVKLIKQELDKYKNAVTELQLLMQSTPATNNRARRELPQFMNYTLNNAQQTNVTLSQNQNQNFLGFLLGVGSAIASGVAVSKVLHLEGEVNKIKSALLSTNKAVVSLSNGVSVLTSKVLDLKNYIDKQLLPIVNKQSCSISNIETVIEFQQKNNRLLEITREFSVNAGVTTPVSTYMLTNSELLSLINDMPITNDQKKLMSNNVQIVRQQSYSIMSIIKEEVLAYVVQLPLYGVIDTPCWKLHTSPLCTTNTKEGSNICLTRTDRGWYCDNAGSVSFFPQAETCKVQSNRVFCDTMNSLTLPSEVNLCNVDIFNPKYDCKIMTSKTDVSSSVITSLGAIVSCYGKTKCTASNKNRGIIKTFSNGCDYVSNKGVDTVSVGNTLYYVNKQEGKSLYVKGEPIINFYDPLVFPSDEFDASISQVNEKINQSLAFIRKSDELLHNVNAGKSTTNGGSAGSGHHHHHH

SEQ ID NO: 67 - protein, 528 aa, synthetic construct
  REGION 1..528: note = Description of Artificial Sequence: Syntheticpolypeptide
MELLILKANAITTILTAVTFCFASGQNITEEFYQSTCSAVSKGYLSALRTGWYTSVITIELSNIKENKCNGTDAKVKLIKQELDKYKNAVTELQLLMQSTPATNNRARRELPRFMNYTLNNAKKTNVTLSKKRKRRSAIASGVAVSKVLHLEGEVNKIKSALLSTNKAVVSLSNGVSVLTSKVLDLKNYIDKQLLPIVNKQSCSISNIETVIEFQQKNNRLLEITREFSVNAGVTTPVSTYMLTNSELLSLINDMPITNDQKKLMSNNVQIVRQQSYSIMSIIKEEVLAYVVQLPLYGVIDTPCWKLHTSPLCTTNTKEGSNICLTRTDRGWYCDNAGSVSFFPQAETCKVQSNRVFCDTMNSLTLPSEVNLCNVDIFNPKYDCKIMTSKTDVSSSVITSLGAIVSCYGKTKCTASNKNRGIIKTFSNGCDYVSNKGVDTVSVGNTLYYVNKQEGKSLYVKGEPIINFYDPLVFPSDEFDASISQVNEKINQSLAFIRKSDELLHNVNAGKSTTNGGSAGSGHHHHHH

SEQ ID NO: 68 - protein, 531 aa, synthetic construct
  REGION 1..531: note = Description of Artificial Sequence: Syntheticpolypeptide
MELLILKANAITTILTAVTFCFASGQNITEEFYQSTCSAVSKGYLSALRTGWYTSVITIELSNIKENKCNGTDAKVKLIKQELDKYKNAVTELQLLMQSTPATNNRARRELPRFMNYTLNNAKKTNVTLSKKRKRRGVGSAIASGVAVSKVLHLEGEVNKIKSALLSTNKAVVSLSNGVSVLTSKVLDLKNYIDKQLLPIVNKQSCSISNIETVIEFQQKNNRLLEITREFSVNAGVTTPVSTYMLTNSELLSLINDMPITNDQKKLMSNNVQIVRQQSYSIMSIIKEEVLAYVVQLPLYGVIDTPCWKLHTSPLCTTNTKEGSNICLTRTDRGWYCDNAGSVSFFPQAETCKVQSNRVFCDTMNSLTLPSEVNLCNVDIFNPKYDCKIMTSKTDVSSSVITSLGAIVSCYGKTKCTASNKNRGIIKTFSNGCDYVSNKGVDTVSVGNTLYYVNKQEGKSLYVKGEPIINFYDPLVFPSDEFDASISQVNEKINQSLAFIRKSDELLHNVNAGKSTTNGGSAGSGHHHHHH

SEQ ID NO: 69 - protein, 537 aa, synthetic construct
  REGION 1..537: note = Description of Artificial Sequence: Syntheticpolypeptide
MELLILKANAITTILTAVTFCFASGQNITEEFYQSTCSAVSKGYLSALRTGWYTSVITIELSNIKENKCNGTDAKVKLIKQELDKYKNAVTELQLLMQSTPATNNQAQNELPQFMNYTLNNAQQTNVTLSQNQNQNFLGFLLGVGSAIASGVAVSKVLHLEGEVNKIKSALLSTNKAVVSLSNGVSVLTSKVLDLKNYIDKQLLPIVNKQSCSISNIETVIEFQQKNNRLLEITREFSVNAGVTTPVSTYMLTNSELLSLINDMPITNDQKKLMSNNVQIVRQQSYSIMSIIKEEVLAYVVQLPLYGVIDTPCWKLHTSPLCTTNTKEGSNICLTRTDRGWYCDNAGSVSFFPQAETCKVQSNRVFCDTMNSLTLPSEVNLCNVDIFNPKYDCKIMTSKTDVSSSVITSLGAIVSCYGKTKCTASNKNRGIIKTFSNGCDYVSNKGVDTVSVGNTLYYVNKQEGKSLYVKGEPIINFYDPLVFPSDEFDASISQVNEKINQSLAFIRKSDELLHNVNAGKSTTNGGSAGSGHHHHHH

SEQ ID NO: 70 - protein, 524 aa, synthetic construct
  REGION 1..524: note = Description of Artificial Sequence: Syntheticpolypeptide
MELLILKANAITTILTAVTFCFASGQNITEEFYQSTCSAVSKGYLSALRTGWYTSVITIELSNIKENKCNGTDAKVKLIKQELDKYKNAVTELQLLMQSTPATNNQAQNELPQFMNYTLNNAQQTNVTLSQNQNQNFLGFLLGVGSAIASGVAVSKVLHLEGEVNKIKSALLSTNKAVVSLSNGVSVLTSKVLDLKNYIDKQLLPIVNKQSCSISNIETVIEFQQKNNRLLEITREFSVNAGVTTPVSTYMLTNSELLSLINDMPITNDQKKLMSNNVQIVRQQSYSIMSIIKEEVLAYVVQLPLYGVIDTPCWKLHTSPLCTTNTKEGSNICLTRTDRGWYCDNAGSVSFFPQAETCKVQSNRVFCDTMNSLTLPSEVNLCNVDIFNPKYDCKIMTSKTDVSSSVITSLGAIVSCYGKTKCTASNKNRGIIKTFSNGCDYVSNKGVDTVSVGNTLYYVNKQEGKSLYVKGEPIINFYDPLVFPSDEFDASISQVNEKINQSLAFIRKSDELLHNVNAGKSTTN

SEQ ID NO: 71 - protein, 501 aa, synthetic construct
  REGION 1..501: note = Description of Artificial Sequence: Syntheticpolypeptide
MELLILKANAITTILTAVTFCFASGQNITEEFYQSTCSAVSKGYLSALRTGWYTSVITIELSNIKENKCNGTDAKVKLIKQELDKYKNAVTELQLLMQSTPATNNRARQQQQRFLGFLLGVGSAIASGVAVSKVLHLEGEVNKIKSALLSTNKAVVSLSNGVSVLTSKVLDLKNYIDKQLLPIVNKQSCSISNIETVIEFQQKNNRLLEITREFSVNAGVTTPVSTYMLTNSELLSLINDMPITNDQKKLMSNNVQIVRQQSYSIMSIIKEEVLAYVVQLPLYGVIDTPCWKLHTSPLCTTNTKEGSNICLTRTDRGWYCDNAGSVSFFPQAETCKVQSNRVFCDTMNSLTLPSEVNLCNVDIFNPKYDCKIMTSKTDVSSSVITSLGAIVSCYGKTKCTASNKNRGIIKTFSNGCDYVSNKGVDTVSVGNTLYYVNKQEGKSLYVKGEPIINFYDPLVFPSDEFDASISQVNEKINQSLAFIRKSDELLHNVNAGKSTTN

SEQ ID NO: 72 - DNA, 18 bp, synthetic construct
  misc_feature 1..18: note = Description of Artificial Sequence: Syntheticprimer
  source 1..18: mol_type = other DNA
ttggatctgcaatcgcca

SEQ ID NO: 73 - DNA, 27 bp, synthetic construct
  misc_feature 1..27: note = Description of Artificial Sequence: Syntheticprimer
  source 1..27: mol_type = other DNA
cttttgatcttgttcacttctccttct

SEQ ID NO: 74 - DNA, 29 bp, synthetic construct
  misc_feature 1..29: note = Description of Artificial Sequence: Syntheticprobe
  source 1..29: mol_type = other DNA
tggcactgctgtatctaaggtcctgcact

SEQ ID NO: 75 - protein, 4 aa, synthetic construct
  REGION 1..4: note = Description of Artificial Sequence: Syntheticpeptide
LVPR

SEQ ID NO: 76 - protein, 5 aa, synthetic construct
  REGION 1..5: note = Description of Artificial Sequence: Syntheticpeptide
DDDDK

SEQ ID NO: 77 - protein, 4 aa, synthetic construct
  REGION 1..4: note = Description of Artificial Sequence: Syntheticpeptide
RARK

SEQ ID NO: 78 - protein, 4 aa, synthetic construct
  REGION 1..4: note = Description of Artificial Sequence: Syntheticpeptide
RARQ

SEQ ID NO: 79 - protein, 4 aa, synthetic construct
  REGION 1..4: note = Description of Artificial Sequence: Syntheticpeptide
QAQN

SEQ ID NO: 80 - protein, 4 aa, synthetic construct
  REGION 1..4: note = Description of Artificial Sequence: Syntheticpeptide
IEGR

SEQ ID NO: 81 - protein, 4 aa, synthetic construct
  REGION 1..4: note = Description of Artificial Sequence: Syntheticpeptide
RKKK

SEQ ID NO: 82 - protein, 4 aa, synthetic construct
  REGION 1..4: note = Description of Artificial Sequence: Syntheticpeptide
QNQN

SEQ ID NO: 83 - protein, 4 aa, synthetic construct
  REGION 1..4: note = Description of Artificial Sequence: Syntheticpeptide
QQQR

SEQ ID NO: 84 - protein, 537 aa, synthetic construct
  REGION 1..537: note = Description of Artificial Sequence: Syntheticpolypeptide
MELLILKANAITTILTAVTFCFASGQNITEEFYQSTCSAVSKGYLSALRTGWYTSVITIELSNIKENKCNGTDAKVKLIKQELDKYKNAVTELQLLMQSTPATNNRARRELPRFMNYTLNNAKKTNVTLSKKRKRRFLGFLLGVGSAIASGVAVSKVLHLEGEVNKIKSALLSTNKAVVSLSNGVSVLTSKVLDLKNYIDKQLLPIVNKQSCSISNIETVIEFQQKNNRLLEITREFSVNAGVTTPVSTYMLTNSELLSLINDMPITNDQKKLMSNNVQIVRQQSYSIMSIIKEEVLAYVVQLPLYGVIDTPCWKLHTSPLCTTNTKEGSNICLTRTDRGWYCDNAGSVSFFPQAETCKVQSNRVFCDTMNSLTLPSEVNLCNVDIFNPKYDCKIMTSKTDVSSSVITSLGAIVSCYGKTKCTASNKNRGIIKTFSNGCDYVSNKGVDTVSVGNTLYYVNKQEGKSLYVKGEPIINFYDPLVFPSDEFDASISQVNEKINQSLAFIRKSDELLHNVNAGKSTTNGGSAGSGHHHHHH

SEQ ID NO: 85 - protein, 537 aa, synthetic construct; identical to SEQ ID NO: 66
  REGION 1..537: note = Description of Artificial Sequence: Syntheticpolypeptide

SEQ ID NO: 86 - protein, 516 aa, synthetic construct
  REGION 1..516: note = Description of Artificial Sequence: Syntheticpolypeptide
MELLILKANAITTILTAVTFCFASGQNITEEFYQSTCSAVSKGYLSALRTGWYTSVITIELSNIKENKCNGTDAKVKLIKQELDKYKNAVTELQLLMQSTPATNNRARQQNQQQRFLGFLLGVGSAIASGVAVSKVLHLEGEVNKIKSALLSTNKAVVSLSNGVSVLTSKVLDLKNYIDKQLLPIVNKQSCSISNIETVIEFQQKNNRLLEITREFSVNAGVTTPVSTYMLTNSELLSLINDMPITNDQKKLMSNNVQIVRQQSYSIMSIIKEEVLAYVVQLPLYGVIDTPCWKLHTSPLCTTNTKEGSNICLTRTDRGWYCDNAGSVSFFPQAETCKVQSNRVFCDTMNSLTLPSEVNLCNVDIFNPKYDCKIMTSKTDVSSSVITSLGAIVSCYGKTKCTASNKNRGIIKTFSNGCDYVSNKGVDTVSVGNTLYYVNKQEGKSLYVKGEPIINFYDPLVFPSDEFDASISQVNEKINQSLAFIRKSDELLHNVNAGKSTTNGGSAGSGHHHHHH

SEQ ID NO: 87 - protein, 537 aa, synthetic construct; identical to SEQ ID NO: 65
  REGION 1..537: note = Description of Artificial Sequence: Syntheticpolypeptide

SEQ ID NO: 88 - protein, 537 aa, synthetic construct
  REGION 1..537: note = Description of Artificial Sequence: Syntheticpolypeptide
MELLILKANAITTILTAVTFCFASGQNITEEFYQSTCSAVSKGYLSALRTGWYTSVITIELSNIKENKCNGTDAKVKLIKQELDKYKNAVTELQLLMQSTPATNNQAQNELQRFMNYTLNNANNTNVTLSQNQNQNFLGFLLGVGSAIASGVAVSKVLHLEGEVNKIKSALLSTNKAVVSLSNGVSVLTSKVLDLKNYIDKQLLPIVNKQSCSISNIETVIEFQQKNNRLLEITREFSVNAGVTTPVSTYMLTNSELLSLINDMPITNDQKKLMSNNVQIVRQQSYSIMSIIKEEVLAYVVQLPLYGVIDTPCWKLHTSPLCTTNTKEGSNICLTRTDRGWYCDNAGSVSFFPQAETCKVQSNRVFCDTMNSLTLPSEVNLCNVDIFNPKYDCKIMTSKTDVSSSVITSLGAIVSCYGKTKCTASNKNRGIIKTFSNGCDYVSNKGVDTVSVGNTLYYVNKQEGKSLYVKGEPIINFYDPLVFPSDEFDASISQVNEKINQSLAFIRKSDELLHNVNAGKSTTNGGSAGSGHHHHHH

SEQ ID NO: 89 - protein, 537 aa, synthetic construct; identical to SEQ ID NO: 69
  REGION 1..537: note = Description of Artificial Sequence: Syntheticpolypeptide

SEQ ID NO: 90 - protein, 13 aa, synthetic construct
  REGION 1..13: note = Description of Artificial Sequence: Syntheticpeptide
GGSAGSGHHHHHH

SEQ ID NO: 91 - protein, 45 aa, synthetic construct
  REGION 1..45: note = Description of Artificial Sequence: Syntheticpolypeptide
TPATNNRARRELPRFMNYTLNNAKKTNVTLSKKRKRRGVGSAIAS

SEQ ID NO: 92 - protein, 51 aa, synthetic construct
  REGION 1..51: note = Description of Artificial Sequence: Syntheticpolypeptide
TPATNNQAQNELPQFMNYTLNNAQQTNVTLSQNQNQNFLGFLLGVGSAIAS

SEQ ID NO: 93 - protein, 537 aa, synthetic construct; identical to SEQ ID NO: 69
  REGION 1..537: note = Description of Artificial Sequence: Syntheticpolypeptide

SEQ ID NO: 94 - protein, 37 aa, Human respiratory syncytial virus
FDASISQVNEKINQSLAFIRKSDELLHHVNAGKSTTN

SEQ ID NO: 95 - protein, 52 aa, synthetic construct
  REGION 1..52: note = Description of Artificial Sequence: Syntheticpolypeptide
FDASISQINEKINQSIAFIRKIDELLHHINAGKSTTNGSGSGDDDDKGSGSG

SEQ ID NO: 96 - protein, 71 aa, synthetic construct
  REGION 1..71: note = Description of Artificial Sequence: Syntheticpolypeptide
FDASISQVNEKINQSLAFIRKSDELLHNVNDKIEEILSKIYHIENEIARIKKLIGEGSGSGDDDDKGSGSG

SEQ ID NO: 97 - protein, 51 aa, synthetic construct
  REGION 1..51: note = Description of Artificial Sequence: Syntheticpolypeptide
FDASISQINEKINQILAFIRKIDELLHHINAGKSTTNGSGSGIEGRGSGSG

SEQ ID NO: 98 - protein, 70 aa, synthetic construct
  REGION 1..70: note = Description of Artificial Sequence: Syntheticpolypeptide
FDASISQVNEKINQSLAFIRKSDELLHHVNDKIEEILSKIYHIENEIARIKKLIGEGSGSGIEGRGSGSG

SEQ ID NO: 99 - protein, 51 aa, synthetic construct
  REGION 1..51: note = Description of Artificial Sequence: Syntheticpolypeptide
FDASISQINEKINQILAFIRKIDELLHNINAGKSTTNGSGSGLVPRGSGSG

SEQ ID NO: 100 - protein, 70 aa, synthetic construct
  REGION 1..70: note = Description of Artificial Sequence: Syntheticpolypeptide
FDASISQVNEKINQSLAFIRKSDELLHNVNDKIEEILSKIYHIENEIARIKKLIGEGSGSGLVPRGSGSG

SEQ ID NO: 101 - DNA, 12463 bp, synthetic construct
  misc_feature 1..12463: note = Description of Artificial Sequence: Syntheticpolynucleotide
  source 1..12463: mol_type = other DNA
ataggcggcgcatgagagaagcccagaccaattacctacccaaaatggagaaagttcacgttgacatcgaggaagacagcccattcctcagagctttgcagcggagcttcccgcagtttgaggtagaagccaagcaggtcactgataatgaccatgctaatgccagagcgttttcgcatctggcttcaaaactgatcgaaacggaggtggacccatccgacacgatccttgacattggaagtgcgcccgcccgcagaatgtattctaagcacaagtatcattgtatctgtccgatgagatgtgcggaagatccggacagattgtataagtatgcaactaagctgaagaaaaactgtaaggaaataactgataaggaattggacaagaaaatgaaggagctcgccgccgtcatgagcgaccctgacctggaaactgagactatgtgcctccacgacgacgagtcgtgtcgctacgaagggcaagtcgctgtttaccaggatgtatacgcggttgacggaccgacaagtctctatcaccaagccaataagggagttagagtcgcctactggataggctttgacaccaccccttttatgtttaagaacttggctggagcatatccatcatactctaccaactgggccgacgaaaccgtgttaacggctcgtaacataggcctatgcagctctgacgttatggagcggtcacgtagagggatgtccattcttagaaagaagtatttgaaaccatccaacaatgttctattctctgttggctcgaccatctaccacgagaagagggacttactgaggagctggcacctgccgtctgtatttcacttacgtggcaagcaaaattacacatgtcggtgtgagactatagttagttgcgacgggtacgtcgttaaaagaatagctatcagtccaggcctgtatgggaagccttcaggctatgctgctacgatgcaccgcgagggattcttgtgctgcaaagtgacagacacattgaacggggagagggtctcttttcccgtgtgcacgtatgtgccagctacattgtgtgaccaaatgactggcatactggcaacagatgtcagtgcggacgacgcgcaaaaactgctggttgggctcaaccagcgtatagtcgtcaacggtcgcacccagagaaacaccaataccatgaaaaattaccttttgcccgtagtggcccaggcatttgctaggtgggcaaaggaatataaggaagatcaagaagatgaaaggccactaggactacgagatagacagttagtcatggggtgttgttgggcttttagaaggcacaagataacatctatttataagcgcccggatacccaaaccatcatcaaagtgaacagcgatttccactcattcgtgctgcccaggataggcagtaacacattggagatcgggctgagaacaagaatcaggaaaatgttagaggagcacaaggagccgtcacctctcattaccgccgaggacgtacaagaagctaagtgcgcagccgatgaggctaaggaggtgcgtgaagccgaggagttgcgcgcagctctaccacctttggcagctgatgttgaggagcccactctggaagccgatgtagacttgatgttacaagaggctggggccggctcagtggagacacctcgtggcttgataaaggttaccagctacgatggcgaggacaagatcggctcttacgctgtgctttctccgcaggctgtactcaagagtgaaaaattatcttgcatccaccctctcgctgaacaagtcatagtgataacacactctggccgaaaagggcgttatgccgtggaaccataccatggtaaagtagtggtgccagagggacatgcaatacccgtccaggactttcaagctctgagtgaaagtgccaccattgtgtacaacgaacgtgagttcgtaaacaggtacctgcaccatattgccacacatggaggagcgctgaacactgatgaagaatattacaaaactgtcaagcccagcgagcacgacggcgaatacctgtacgacatcgacaggaaacagtgcgtcaagaaagaactagtcactgggctagggctcacaggcgagctggtggatcctcccttccatgaattcgcctacgagagtctgagaacacgaccagccgctccttaccaagtaccaaccataggggtgtatggcgtgccaggatcaggcaagtctggcatcattaaaagcgcagtcaccaaaaaagatctagtggtgagcgccaagaaagaaaactgtgcagaaattataagggacgtcaagaaaatgaaagggctggacgtcaatgccagaactgtggactcagtgctcttgaatggatgcaaacaccccgtagagaccctgtatattgacgaagcttttgcttgtcatgcaggtactctcagagcgctcatagccattataagacctaaaaaggcagtgctctgcggggatcccaaacagtgcggtttttttaacatgatgtgcctgaaagtgcattttaaccacgagatttgcacacaagtcttccacaaaagcatctctcgccgttgcactaaatctgtgacttcggtcgtctcaaccttgttttacgacaaaaaaatgagaacgacgaatccgaaagagactaagattgtgattgacactaccggcagtaccaaacctaagcaggacgatctcattctcacttgtttcagagggtgggtgaagcagttgcaaatagattacaaaggcaacgaaataatgacggcagctgcctctcaagggctgacccgtaaaggtgtgtatgccgttcggtacaaggtgaatgaaaatcctctgtacgcacccacctcagaacatgtgaacgtcctactgacccgcacggaggaccgcatcgtgtggaaaacactagccggcgacccatggataaaaacactgactgccaagtaccctgggaatttcactgccacgatagaggagtggcaagcagagcatgatgccatcatgaggcacatcttggagagaccggaccctaccgacgtcttccagaataaggcaaacgtgtgttgggccaaggctttagtgccggtgctgaagaccgctggcatagacatgaccactgaacaatggaacactgtggattattttgaaacggacaaagctcactcagcagagatagtattgaaccaactatgcgtgaggttctttggactcgatctggactccggtctattttctgcacccactgttccgttatccattaggaataatcactgggataactccccgtcgcctaacatgtacgggctgaataaagaagtggtccgtcagctctctcgcaggtacccacaactgcctcgggcagttgccactggaagagtctatgacatgaacactggtacactgcgcaattatgatccgcgcataaacctagtacctgtaaacagaagactgcctcatgctttagtcctccaccataatgaacacccacagagtgacttttcttcattcgtcagcaaattgaagggcagaactgtcctggtggtcggggaaaagttgtccgtcccaggcaaaatggttgactggttgtcagaccggcctgaggctaccttcagagctcggctggatttaggcatcccaggtgatgtgcccaaatatgacataatatttgttaatgtgaggaccccatataaataccatcactatcagcagtgtgaagaccatgccattaagcttagcatgttgaccaagaaagcttgtctgcatctgaatcccggcggaacctgtgtcagcataggttatggttacgctgacagggccagcgaaagcatcattggtgctatagcgcggcagttcaagttttcccgggtatgcaaaccgaaatcctcacttgaagagacggaagttctgtttgtattcattgggtacgatcgcaaggcccgtacgcacaatccttacaagctttcatcaaccttgaccaacatttatacaggttccagactccacgaagccggatgtgcaccctcatatcatgtggtgcgaggggatattgccacggccaccgaaggagtgattataaatgctgctaacagcaaaggacaacctggcggaggggtgtgcggagcgctgtataagaaattcccggaaagcttcgatttacagccgatcgaagtaggaaaagcgcgactggtcaaaggtgcagctaaacatatcattcatgccgtaggaccaaacttcaacaaagtttcggaggttgaaggtgacaaacagttggcagaggcttatgagtccatcgctaagattgtcaacgataacaattacaagtcagtagcgattccactgttgtccaccggcatcttttccgggaacaaagatcgactaacccaatcattgaaccatttgctgacagctttagacaccactgatgcagatgtagccatatactgcagggacaagaaatgggaaatgactctcaaggaagcagtggctaggagagaagcagtggaggagatatgcatatccgacgactcttcagtgacagaacctgatgcagagctggtgagggtgcatccgaagagttctttggctggaaggaagggctacagcacaagcgatggcaaaactttctcatatttggaagggaccaagtttcaccaggcggccaaggatatagcagaaattaatgccatgtggcccgttgcaacggaggccaatgagcaggtatgcatgtatatcctcggagaaagcatgagcagtattaggtcgaaatgccccgtcgaagagtcggaagcctccacaccacctagcacgctgccttgcttgtgcatccatgccatgactccagaaagagtacagcgcctaaaagcctcacgtccagaacaaattactgtgtgctcatcctttccattgccgaagtatagaatcactggtgtgcagaagatccaatgctcccagcctatattgttctcaccgaaagtgcctgcgtatattcatccaaggaagtatctcgtggaaacaccaccggtagacgagactccggagccatcggcagagaaccaatccacagaggggacacctgaacaaccaccacttataaccgaggatgagaccaggactagaacgcctgagccgatcatcatcgaagaggaagaagaggatagcataagtttgctgtcagatggcccgacccaccaggtgctgcaagtcgaggcagacattcacgggccgccctctgtatctagctcatcctggtccattcctcatgcatccgactttgatgtggacagtttatccatacttgacaccctggagggagctagcgtgaccagcggggcaacgtcagccgagactaactcttacttcgcaaagagtatggagtttctggcgcgaccggtgcctgcgcctcgaacagtattcaggaaccctccacatcccgctccgcgcacaagaacaccgtcacttgcacccagcagggcctgctcgagaaccagcctagtttccaccccgccaggcgtgaatagggtgatcactagagaggagctcgaggcgcttaccccgtcacgcactcctagcaggtcggtctcgagaaccagcctggtctccaacccgccaggcgtaaatagggtgattacaagagaggagtttgaggcgttcgtagcacaacaacaatgacggtttgatgcgggtgcatacatcttttcctccgacaccggtcaagggcatttacaacaaaaatcagtaaggcaaacggtgctatccgaagtggtgttggagaggaccgaattggagatttcgtatgccccgcgcctcgaccaagaaaaagaagaattactacgcaagaaattacagttaaatcccacacctgctaacagaagcagataccagtccaggaaggtggagaacatgaaagccataacagctagacgtattctgcaaggcctagggcattatttgaaggcagaaggaaaagtggagtgctaccgaaccctgcatcctgttcctttgtattcatctagtgtgaaccgtgccttttcaagccccaaggtcgcagtggaagcctgtaacgccatgttgaaagagaactttccgactgtggcttcttactgtattattccagagtacgatgcctatttggacatggttgacggagcttcatgctgcttagacactgccagtttttgccctgcaaagctgcgcagctttccaaagaaacactcctatttggaacccacaatacgatcggcagtgccttcagcgatccagaacacgctccagaacgtcctggcagctgccacaaaaagaaattgcaatgtcacgcaaatgagagaattgcccgtattggattcggcggcctttaatgtggaatgcttcaagaaatatgcgtgtaataatgaatattgggaaacgtttaaagaaaaccccatcaggcttactgaagaaaacgtggtaaattacattaccaaattaaaaggaccaaaagctgctgctctttttgcgaagacacataatttgaatatgttgcaggacataccaatggacaggtttgtaatggacttaaagagagacgtgaaagtgactccaggaacaaaacatactgaagaacggcccaaggtacaggtgatccaggctgccgatccgctagcaacagcgtatctgtgcggaatccaccgagagctggttaggagattaaatgcggtcctgcttccgaacattcatacactgtttgatatgtcggctgaagactttgacgctattatagccgagcacttccagcctggggattgtgttctggaaactgacatcgcgtcgtttgataaaagtgaggacgacgccatggctctgaccgcgttaatgattctggaagacttaggtgtggacgcagagctgttgacgctgattgaggcggctttcggcgaaatttcatcaatacatttgcccactaaaactaaatttaaattcggagccatgatgaaatctggaatgttcctcacactgtttgtgaacacagtcattaacattgtaatcgcaagcagagtgttgagagaacggctaaccggatcaccatgtgcagcattcattggagatgacaatatcgtgaaaggagtcaaatcggacaaattaatggcagacaggtgcgccacctggttgaatatggaagtcaagattatagatgctgtggtgggcgagaaagcgccttatttctgtggagggtttattttgtgtgactccgtgaccggcacagcgtgccgtgtggcagaccccctaaaaaggctgtttaagcttggcaaacctctggcagcagacgatgaacatgatgatgacaggagaagggcattgcatgaagagtcaacacgctggaaccgagtgggtattctttcagagctgtgcaaggcagtagaatcaaggtatgaaaccgtaggaacttccatcatagttatggccatgactactctagctagcagtgttaaatcattcagctacctgagaggggcccctataactctctacggctaacctgaatggactacgacatagtctagtcgacgccaccatggaactgctgatcctgaaggccaacgccatcaccaccatcctgaccgccgtgaccttctgcttcgccagcggccagaacatcaccgaggaattctaccagagcacctgcagcgccgtgagcaagggctacctgagcgccctgcggaccggctggtacaccagcgtgatcaccatcgagctgtccaacatcaaagaaaacaagtgcaacggcaccgacgccaaggtgaaactgatcaagcaggaactggacaagtacaagaacgccgtgaccgagctgcagctgctgatgcagagcacccccgccaccaacaaccgggccagaagagagctgccccggttcatgaactacaccctgaacaacgccaagaaaaccaacgtgaccctgagcaagaagcggaagcggcggttcctgggcttcctgctgggcgtgggcagcgccatcgccagcggggtggccgtgtccaaggtgctgcacctggaaggcgaggtgaacaagatcaagtccgccctgctgtccaccaacaaggccgtggtgtccctgagcaacggcgtgagcgtgctgaccagcaaggtgctggatctgaagaactacatcgacaagcagctgctgcccatcgtgaacaagcagagctgcagcatcagcaacatcgagaccgtgatcgagttccagcagaagaacaaccggctgctggaaatcacccgggagttcagcgtgaacgccggcgtgaccacccccgtgagcacctacatgctgaccaacagcgagctgctgtccctgatcaatgacatgcccatcaccaacgaccagaaaaagctgatgagcaacaacgtgcagatcgtgcggcagcagagctactccatcatgagcatcatcaaagaagaggtgctggcctacgtggtgcagctgcccctgtacggcgtgatcgacaccccctgctggaagctgcacaccagccccctgtgcaccaccaacaccaaagagggcagcaacatctgcctgacccggaccgaccggggctggtactgcgacaacgccggcagcgtgagcttcttcccccaagccgagacctgcaaggtgcagagcaaccgggtgttctgcgacaccatgaacagcctgaccctgccctccgaggtgaacctgtgcaacgtggacatcttcaaccccaagtacgactgcaagatcatgacctccaagaccgacgtgagcagctccgtgatcacctccctgggcgccatcgtgagctgctacggcaagaccaagtgcaccgccagcaacaagaaccggggcatcatcaagaccttcagcaacggctgcgactacgtgagcaacaagggcgtggacaccgtgagcgtgggcaacacactgtactacgtgaataagcaggaaggcaagagcctgtacgtgaagggcgagcccatcatcaacttctacgaccccctggtgttccccagcgacgagttcgacgccagcatcagccaggtcaacgagaagatcaaccagagcctggccttcatccggaagagcgacgagctgctgcacaatgtgaatgccggcaagagcaccaccaatatcatgatcaccacaatcatcatcgtgatcattgtgatcctgctgtctctgattgccgtgggcctgctgctgtactgcaaggcccgcagcacccctgtgaccctgtccaaggaccagctgtccggcatcaacaatatcgccttctccaactgaagtctagacggcgcgcccacccagcggccgcatacagcagcaattggcaagctgcttacatagaactcgcggcgattggcatgccgccttaaaatttttattttatttttcttttcttttccgaatcggattttgtttttaatatttcaaaaaaaaaaaaaaaaaaaaaaaaaaaaaaaaaaagggtcggcatggcatctccacctcctcgcggtccgacctgggcatccgaaggaggacgcacgtccactcggatggctaagggagagccacgtttaaaccagctccaattcgccctatagtgagtcgtattacgcgcgctcactggccgtcgttttacaacgtcgtgactgggaaaaccctggcgttacccaacttaatcgccttgcagcacatccccctttcgccagctggcgtaatagcgaagaggcccgcaccgatcgcccttcccaacagttgcgcagcctgaatggcgaatgggacgcgccctgtagcggcgcattaagcgcggcgggtgtggtggttacgcgcagcgtgaccgctacacttgccagcgccctagcgcccgctcctttcgctttcttcccttcctttctcgccacgttcgccggctttccccgtcaagctctaaatcgggggctccctttagggttccgatttagtgctttacggcacctcgaccccaaaaaacttgattagggtgatggttcacgtagtgggccatcgccctgatagacggtttttcgccctttgacgttggagtccacgttctttaatagtggactcttgttccaaactggaacaacactcaaccctatctcggtctattcttttgatttataagggattttgccgatttcggcctattggttaaaaaatgagctgatttaacaaaaatttaacgcgaattttaacaaaatattaacgcttacaatttaggtggcacttttcggggaaatgtgcgcggaacccctatttgtttatttttctaaatacattcaaatatgtatccgctcatgagacaataaccctgataaatgcttcaataatattgaaaaaggaagagtatgagtattcaacatttccgtgtcgcccttattcccttttttgcggcattttgccttcctgtttttgctcacccagaaacgctggtgaaagtaaaagatgctgaagatcagttgggtgcacgagtgggttacatcgaactggatctcaacagcggtaagatccttgagagttttcgccccgaagaacgttttccaatgatgagcacttttaaagttctgctatgtggcgcggtattatcccgtattgacgccgggcaagagcaactcggtcgccgcatacactattctcagaatgacttggttgagtactcaccagtcacagaaaagcatcttacggatggcatgacagtaagagaattatgcagtgctgccataaccatgagtgataacactgcggccaacttacttctgacaacgatcggaggaccgaaggagctaaccgcttttttgcacaacatgggggatcatgtaactcgccttgatcgttgggaaccggagctgaatgaagccataccaaacgacgagcgtgacaccacgatgcctgtagcaatggcaacaacgttgcgcaaactattaactggcgaactacttactctagcttcccggcaacaattaatagactggatggaggcggataaagttgcaggaccacttctgcgctcggcccttccggctggctggtttattgctgataaatctggagccggtgagcgtgggtctcgcggtatcattgcagcactggggccagatggtaagccctcccgtatcgtagttatctacacgacggggagtcaggcaactatggatgaacgaaatagacagatcgctgagataggtgcctcactgattaagcattggtaactgtcagaccaagtttactcatatatactttagattgatttaaaacttcatttttaatttaaaaggatctaggtgaagatcctttttgataatctcatgaccaaaatcccttaacgtgagttttcgttccactgagcgtcagaccccgtagaaaagatcaaaggatcttcttgagatcctttttttctgcgcgtaatctgctgcttgcaaacaaaaaaaccaccgctaccagcggtggtttgtttgccggatcaagagctaccaactctttttccgaaggtaactggcttcagcagagcgcagataccaaatactgttcttctagtgtagccgtagttaggccaccacttcaagaactctgtagcaccgcctacatacctcgctctgctaatcctgttaccagtggctgctgccagtggcgataagtcgtgtcttaccgggttggactcaagacgatagttaccggataaggcgcagcggtcgggctgaacggggggttcgtgcacacagcccagcttggagcgaacgacctacaccgaactgagatacctacagcgtgagctatgagaaagcgccacgcttcccgaagggagaaaggcggacaggtatccggtaagcggcagggtcggaacaggagagcgcacgagggagcttccagggggaaacgcctggtatctttatagtcctgtcgggtttcgccacctctgacttgagcgtcgatttttgtgatgctcgtcaggggggcggagcctatggaaaaacgccagcaacgcggcctttttacggttcctggccttttgctggccttttgctcacatgttctttcctgcgttatcccctgattctgtggataaccgtattaccgcctttgagtgagctgataccgctcgccgcagccgaacgaccgagcgcagcgagtcagtgagcgaggaagcggaagagcgcccaatacgcaaaccgcctctccccgcgcgttggccgattcattaatgcagctggcacgacaggtttcccgactggaaagcgggcagtgagcgcaacgcaattaatgtgagttagctcactcattaggcaccccaggctttacactttatgctcccggctcgtatgttgtgtggaattgtgagcggataacaatttcacacaggaaacagctatgaccatgattacgccaagcgcgcaattaaccctcactaaagggaacaaaagctgggtaccgggcccacgcgtaatacgactcactatag

SEQ ID NO: 102 - protein, 574 aa, Human respiratory syncytial virus
MELLILKANAITTILTAVTFCFASGQNITEEFYQSTCSAVSKGYLSALRTGWYTSVITIELSNIKENKCNGTDAKVKLIKQELDKYKNAVTELQLLMQSTPATNNRARRELPRFMNYTLNNAKKTNVTLSKKRKRRFLGFLLGVGSAIASGVAVSKVLHLEGEVNKIKSALLSTNKAVVSLSNGVSVLTSKVLDLKNYIDKQLLPIVNKQSCSISNIATVIEFQQKNNRLLEITREFSVNAGVTTPVSTYMLTNSELLSLINDMPITNDQKKLMSNNVQIVRQQSYSIMSIIKEEVLAYVVQLPLYGVIDTPCWKLHTSPLCTTNTKEGSNICLTRTDRGWYCDNAGSVSFFPQAETCKVQSNRVFCDTMNSLTLPSEVNLCNVDIFNPKYDCKIMTSKTDVSSSVITSLGAIVSCYGKTKCTASNKNRGIIKTFSNGCDYVSNKGVDTVSVGNTLYYVNKQEGKSLYVKGEPIINFYDPLVFPSDEFDASISQVNEKINQSLAFIRKSDELLHNVNAGKSTINIMITTIIIVIIVILLSLIAVGLLLYCKARSTPVTLSKDQLSGINNIAFSN

SEQ ID NO: 103 - protein, 574 aa, Human respiratory syncytial virus
MELLIHRLSAIFLTLAINALYLTSSQNITEEFYQSTCSAVSRGYFSALRTGWYTSVITIELSNIKETKCNGTDTKVKLIKQELDKYKNAVTELQLLMQNTPAANNRARREAPQYMNYTINTTKNLNVSISKKRKRRFLGFLLGVGSAIASGIAVSKVLHLEGEVNKIKNALLSTNKAVVSLSNGVSVLTSKVLDLKNYINNQLLPIVNQQSCRISNIGTVIEFQQKNSRLLEINREFSVNAGVTTPLSTYMLTNSELLSLINDMPITNDQKKLMSSNVQIVRQQSYSIMSIIKEEVLAYVVQLPIYGVIDTPCWKLHTSPLCTTNIKEGSNICLTRTDRGWYCDNAGSVSFFPQADTCKVQSNRVFCDTMNSLTLPSEVSLCNTDIFNSKYDCKIMTSKTDISSSVITSLGAIVSCYGKTKCTASNKNRGIIKTFSNGCDYVSNKGVDTVSVGNTLYYVNKLEGKNLYVKGEPIINYYDPLVFPSDEFDASISQVNEKINQSLAFIRRSDELLHNVNTGKSTTNIMITTIIIVIIVVLLSLIAIGLLLYCKAKNTPVTLSKDQLSGINNIAFSK

SEQ ID NO: 104 - protein, 574 aa, Human respiratory syncytial virus
MELLIHRLSAIFLTLAINALYLTSSQNITEEFYQSTCSAVSRGYFSALRTGWYTSVITIELSNIKETKCNGTDTKVKLIKQELDKYKNAVTELQLLMQNTPAANNRARREAPQYMNYTINTTKNLNVSISKKRKRRFLGFLLGVGSAIASGIAVSKVLHLEGEVNKIKNALLSTNKAVVSLSNGVSVLTSKVLDLKNYINNQLLPIVNQQSCRISNIETVIEFQQKNSRLLEINREFSVNAGVTTPLSTYMLTNSELLSLINDMPITNDQKKLMSSNVQIVRQQSYSIMSIIKEEVLAYVVQLPIYGVIDTPCWKLHTSPLCTTNIKEGSNICLTRTDRGWYCDNAGSVSFFPQADTCKVQSNRVFCDTMNSLTLPSEVSLCNTDIFNSKYDCKIMTSKTDISSSVITSLGAIVSCYGKTKCTASNKNRGIIKTFSNGCDYVSNKGVDTVSVGNTLYYVNKLEGKNLYVKGEPIINYYDPLVFPSDEFDASISQVNEKINQSLAFIRRSDELLHNVNTGKSTTNIMITTIIIVIIVVLLSLIAIGLLLYCKAKNTPVTLSKDQLSGINNIAFSK

SEQ ID NO: 105 - protein, 574 aa, Human respiratory syncytial virus
MELLILKANAITTILAAVTFCFASSQNITEEFYQSTCSAVSKGYLSALRTGWYTSVITIELSNIKENKCNGTDAKVKLINQELDKYKNAVTELQLLMQSTTAANNRARRELPRFMNYTLNNTKKTNVTLSKKRKRRFLGFLLGVGSAIASGIAVSKVLHLEGEVNKIKSALLSTNKAVVSLSNGVSVLTSKVLDLKNYIDKQLLPIVNKQSCRISNIETVIEFQQKNNRLLEITREFSVNAGVTTPVSTYMLTNSELLSLINDMPITNDQKKLMSNNVQIVRQQSYSIMSIIKEEVLAYVVQLPLYGVIDTPCWKLHTSPLCTTNTKEGSNICLTRTDRGWYCDNAGSVSFFPQAETCKVQSNRVFCDTMNSLTLPSEVNLCNVDIFNPKYDCKIMTSKTDVSSSVITSLGAIVSCYGKTKCTASNKNRGIIKTFSNGCDYVSNKGVDTVSVGNTLYYVNKQEGKSLYVKGEPIINFYDPLVFPSDEFDASISQVNEKINQSLAFIRKSDELLHHVNAGKSTTNIMITTIIIVIIVILLSLIAVGLLLYCKARSTPVTLSKDQLSGINNIAFSN

SEQ ID NO: 106 - protein, 574 aa, Human respiratory syncytial virus; identical to SEQ ID NO: 2

SEQ ID NO: 107 - protein, 574 aa, synthetic construct
  REGION 1..574: note = Description of Artificial Sequence: Syntheticconsensus sequence
  MOD_RES 4: note = Leu or Pro
  MOD_RES 6: note = His or Leu
  MOD_RES 7: note = Arg or Lys
  MOD_RES 8: note = Leu, Ser or Ala
  MOD_RES 9: note = Ser or Asn
  MOD_RES 12: note = Phe or Thr
  MOD_RES 13: note = Leu or Thr
  MOD_RES 14: note = Thr or Ile
  MOD_RES 16: note = Ala or Thr
  MOD_RES 17: note = Ile, Val or Ala
  MOD_RES 18: note = Asn or Val
  MOD_RES 19: note = Ala or Thr
  MOD_RES 20: note = Leu or Phe
  MOD_RES 21: note = Tyr or Cys
  MOD_RES 22: note = Leu or Phe
  MOD_RES 23: note = Thr or Ala
  MOD_RES 25: note = Ser or Gly
  MOD_RES 42: note = Arg or Lys
  MOD_RES 45: note = Phe or Leu
  MOD_RES 67: note = Thr or Asn
  MOD_RES 74: note = Thr or Ala
  MOD_RES 80: note = Lys or Asn
  MOD_RES 99: note = Asn or Ser
  MOD_RES 101: note = Pro or Thr
  MOD_RES 103: note = Ala or Thr
  MOD_RES 111: note = Ala or Leu
  MOD_RES 113: note = Gln or Arg
  MOD_RES 114: note = Tyr or Phe
  MOD_RES 119: note = Ile or Leu
  MOD_RES 121: note = Thr or Asn
  MOD_RES 122: note = Thr or Ala
  MOD_RES 124: note = Asn or Lys
  MOD_RES 125: note = Leu or Thr
  MOD_RES 128: note = Ser or Thr
  MOD_RES 129: note = Ile or Leu
  MOD_RES 152: note = Ile or Val
  MOD_RES 169: note = Asn or Ser
  MOD_RES 200: note = Asn or Asp
  MOD_RES 201: note = Asn or Lys
  MOD_RES 202: note = Gln or Arg
  MOD_RES 209: note = Gln or Lys
  MOD_RES 213: note = Arg or Ser
  MOD_RES 218: note = Gly, Glu or Ala
  MOD_RES 226: note = Lys or Met
  MOD_RES 228: note = Ser or Asn
  MOD_RES 234: note = Asn or Thr
  MOD_RES 247: note = Leu or Val
  MOD_RES 276: note = Ser or Asn
  MOD_RES 305: note = Ile or Leu
  MOD_RES 326: note = Ile or Thr
  MOD_RES 356: note = Asp or Glu
  MOD_RES 380: note = Ser or Asn
  MOD_RES 384: note = Thr or Val
  MOD_RES 389: note = Ser or Pro
  MOD_RES 402: note = Ile or Val
  MOD_RES 462: note = Leu or Gln
  MOD_RES 466: note = Asn or Ser
  MOD_RES 477: note = Tyr or Phe
  MOD_RES 508: note = Arg or Lys
  MOD_RES 515: note = Asn or His
  MOD_RES 518: note = Thr or Ala
  MOD_RES 523: note = Thr or Ile
  MOD_RES 537: note = Val or Ile
  MOD_RES 544: note = Ile or Val
  MOD_RES 553: note = Lys or Arg
  MOD_RES 554: note = Asn or Ser
  MOD_RES 574: note = Lys or Asn
MELXIXXXXAIXXXLXXXXXXXXSXQNITEEFYQSTCSAVSXGYXSALRTGWYTSVITIELSNIKEXKCNGTDXKVKLIXQELDKYKNAVTELQLLMQXTXAXNNRARREXPXXMNYTXNXXKXXNVXXSKKRKRRFLGFLLGVGSAIASGXAVSKVLHLEGEVNKIKXALLSTNKAVVSLSNGVSVLTSKVLDLKNYIXXXLLPIVNXQSCXISNIXTVIEFQQXNXRLLEIXREFSVNAGVTTPXSTYMLTNSELLSLINDMPITNDQKKLMSXNVQIVRQQSYSIMSIIKEEVLAYVVQLPXYGVIDTPCWKLHTSPLCTTNXKEGSNICLTRTDRGWYCDNAGSVSFFPQAXTCKVQSNRVFCDTMNSLTLPSEVXLCNXDIFNXKYDCKIMTSKTDXSSSVITSLGAIVSCYGKTKCTASNKNRGIIKTFSNGCDYVSNKGVDTVSVGNTLYYVNKXEGKXLYVKGEPIINXYDPLVFPSDEFDASISQVNEKINQSLAFIRXSDELLHXVNXGKSTXNIMITTIIIVIIVXLLSLIAXGLLLYCKAXXTPVTLSKDQLSGINNIAFSX

SEQ ID NO: 108 - protein, 51 aa, Human respiratory syncytial virus
TPATNNRARRELPRFMNYTLNNAKKTNVTLSKKRKRRFLGFLLGVGSAIAS

SEQ ID NO: 109 - protein, 30 aa, synthetic construct
  REGION 1..30: note = Description of Artificial Sequence: Syntheticpolypeptide
TPATNNRARQQNQQQRFLGFLLGVGSAIAS

SEQ ID NO: 110 - protein, 6 aa, synthetic construct
  REGION 1..6: note = Description of Artificial Sequence: Synthetic6xHis tag
HHHHHH

SEQ ID NO: 111 - protein, 100 aa, synthetic construct
  REGION 1..100: note = Description of Artificial Sequence: Syntheticpolypeptide
  REGION 1..100: note = misc_feature - This sequence may encompass 3-100 Lys residues
KKKKKKKKKKKKKKKKKKKKKKKKKKKKKKKKKKKKKKKKKKKKKKKKKKKKKKKKKKKKKKKKKKKKKKKKKKKKKKKKKKKKKKKKKKKKKKKKKKKK

SEQ ID NO: 112 - protein, 50 aa, synthetic construct
  REGION 1..50: note = Description of Artificial Sequence: Syntheticpolypeptide
IMITTIIIVIIVILLSLIAVGLLLYCKARSTPVTLSKDQLSGINNIAFSN